European Patent Application EP 4 386 084 A1, published June 19, 2024. Title: Improved ACE2 fusion proteins. Applicant: FORMYCON AG (DE). Application EP. The sequence listing filed with the application follows.

SEQUENCE LISTING (87 sequences)

SEQ ID NO: 1 - protein, 715 aa, Homo sapiens
  REGION 1..715: note = ACE2 18-732
QSTIEEQAKTFLDKFNHEAEDLFYQSSLASWNYNTNITEENVQNMNNAGDKWSAFLKEQSTLAQMYPLQEIQNLTVKLQLQALQQNGSSVLSEDKSKRLNTILNTMSTIYSTGKVCNPDNPQECLLLEPGLNEIMANSLDYNERLWAWESWRSEVGKQLRPLYEEYVVLKNEMARANHYEDYGDYWRGDYEVNGVDGYDYSRGQLIEDVEHTFEEIKPLYEHLHAYVRAKLMNAYPSYISPIGCLPAHLLGDMWGRFWTNLYSLTVPFGQKPNIDVTDAMVDQAWDAQRIFKEAEKFFVSVGLPNMTQGFWENSMLTDPGNVQKAVCHPTAWDLGKGDFRILMCTKVTMDDFLTAHHEMGHIQYDMAYAAQPFLLRNGANEGFHEAVGEIMSLSAATPKHLKSIGLLSPDFQEDNETEINFLLKQALTIVGTLPFTYMLEKWRWMVFKGEIPKDQWMKKWWEMKREIVGVVEPVPHDETYCDPASLFHVSNDYSFIRYYTRTLYQFQFQEALCQAAKHEGPLHKCDISNSTEAGQKLFNMLRLGKSEPWTLALENVVGAKNMNVRPLLNYFEPLFTWLKDQNKNSFVGWSTDWSPYADQSIKVRISLKSALGDKAYEWNDNEMYLFRSSVAYAMRQYFLKVKNQMILFGEEDVRVANLKPRISFNFFVTAPKNVSDIIPRTEVEKAIRMSRSRINDAFRLNDNSLEFLGIQPTLG

SEQ ID NO: 2 - protein, 216 aa, Homo sapiens
  REGION 1..216: note = Fc portion of human IgG1
PELLGGPSVFLFPPKPKDTLMISRTPEVTCVVVDVSHEDPEVKFNWYVDGVEVHNAKTKPREEQYNSTYRVVSVLTVLHQDWLNGKEYKCKVSNKALPAPIEKTISKAKGQPREPQVYTLPPSRDELTKNQVSLTCLVKGFYPSDIAVEWESNGQPENNYKTTPPVLDSDGSFFLYSKLTVDKSRWQQGNVFSCSVMHEALHNHYTQKSLSLSPGK

SEQ ID NO: 3 - protein, 216 aa, Homo sapiens
  REGION 1..216: note = Fc portion of human IgG4
PEFLGGPSVFLFPPKPKDTLMISRTPEVTCVVVDVSQEDPEVQFNWYVDGVEVHNAKTKPREEQFNSTYRVVSVLTVLHQDWLNGKEYKCKVSNKGLPSSIEKTISKAKGQPREPQVYTLPPSQEEMTKNQVSLTCLVKGFYPSDIAVEWESNGQPENNYKTTPPVLDSDGSFFLYSRLTVDKSRWQEGNVFSCSVMHEALHNHYTQKSLSLSLGK

SEQ ID NO: 4 - protein, 216 aa, synthetic construct
  REGION 1..216: note = IgG4 YTE
PEFLGGPSVFLFPPKPKDTLYITREPEVTCVVVDVSQEDPEVQFNWYVDGVEVHNAKTKPREEQFNSTYRVVSVLTVLHQDWLNGKEYKCKVSNKGLPSSIEKTISKAKGQPREPQVYTLPPSQEEMTKNQVSLTCLVKGFYPSDIAVEWESNGQPENNYKTTPPVLDSDGSFFLYSRLTVDKSRWQEGNVFSCSVMHEALHNHYTQKSLSLSLGK

SEQ ID NO: 5 - protein, 216 aa, synthetic construct
  REGION 1..216: note = IgG4 T256D T307Q
PEFLGGPSVFLFPPKPKDTLMISRDPEVTCVVVDVSQEDPEVQFNWYVDGVEVHNAKTKPREEQFNSTYRVVSVLQVLHQDWLNGKEYKCKVSNKGLPSSIEKTISKAKGQPREPQVYTLPPSQEEMTKNQVSLTCLVKGFYPSDIAVEWESNGQPENNYKTTPPVLDSDGSFFLYSRLTVDKSRWQEGNVFSCSVMHEALHNHYTQKSLSLSLGK

SEQ ID NO: 6 - protein, 216 aa, synthetic construct
  REGION 1..216: note = IgG1 YTE
PELLGGPSVFLFPPKPKDTLYITREPEVTCVVVDVSHEDPEVKFNWYVDGVEVHNAKTKPREEQYNSTYRVVSVLTVLHQDWLNGKEYKCKVSNKALPAPIEKTISKAKGQPREPQVYTLPPSRDELTKNQVSLTCLVKGFYPSDIAVEWESNGQPENNYKTTPPVLDSDGSFFLYSKLTVDKSRWQQGNVFSCSVMHEALHNHYTQKSLSLSPGK

SEQ ID NO: 7 - protein, 216 aa, synthetic construct
  REGION 1..216: note = IgG1 T256D T307Q
PELLGGPSVFLFPPKPKDTLMISRDPEVTCVVVDVSHEDPEVKFNWYVDGVEVHNAKTKPREEQYNSTYRVVSVLQVLHQDWLNGKEYKCKVSNKALPAPIEKTISKAKGQPREPQVYTLPPSRDELTKNQVSLTCLVKGFYPSDIAVEWESNGQPENNYKTTPPVLDSDGSFFLYSKLTVDKSRWQQGNVFSCSVMHEALHNHYTQKSLSLSPGK

SEQ ID NO: 8 - protein, 11 aa, synthetic construct
  REGION 1..11: note = Linker sequence
GGGSGGGSSSG

SEQ ID NO: 9 - protein, 18 aa, Homo sapiens
  REGION 1..18: note = Signal peptide
MKWVTFISLLFLFSSAYS

SEQ ID NO: 10 - protein, 1273 aa, Severe acute respiratory syndrome related coronavirus 2
  REGION 1..1273: note = Spike protein of SARS-CoV2
MFVFLVLLPLVSSQCVNLTTRTQLPPAYTNSFTRGVYYPDKVFRSSVLHSTQDLFLPFFSNVTWFHAIHVSGTNGTKRFDNPVLPFNDGVYFASTEKSNIIRGWIFGTTLDSKTQSLLIVNNATNVVIKVCEFQFCNDPFLGVYYHKNNKSWMESEFRVYSSANNCTFEYVSQPFLMDLEGKQGNFKNLREFVFKNIDGYFKIYSKHTPINLVRDLPQGFSALEPLVDLPIGINITRFQTLLALHRSYLTPGDSSSGWTAGAAAYYVGYLQPRTFLLKYNENGTITDAVDCALDPLSETKCTLKSFTVEKGIYQTSNFRVQPTESIVRFPNITNLCPFGEVFNATRFASVYAWNRKRISNCVADYSVLYNSASFSTFKCYGVSPTKLNDLCFTNVYADSFVIRGDEVRQIAPGQTGKIADYNYKLPDDFTGCVIAWNSNNLDSKVGGNYNYLYRLFRKSNLKPFERDISTEIYQAGSTPCNGVEGFNCYFPLQSYGFQPTNGVGYQPYRVVVLSFELLHAPATVCGPKKSTNLVKNKCVNFNFNGLTGTGVLTESNKKFLPFQQFGRDIADTTDAVRDPQTLEILDITPCSFGGVSVITPGTNTSNQVAVLYQDVNCTEVPVAIHADQLTPTWRVYSTGSNVFQTRAGCLIGAEHVNNSYECDIPIGAGICASYQTQTNSPRRARSVASQSIIAYTMSLGAENSVAYSNNSIAIPTNFTISVTTEILPVSMTKTSVDCTMYICGDSTECSNLLLQYGSFCTQLNRALTGIAVEQDKNTQEVFAQVKQIYKTPPIKDFGGFNFSQILPDPSKPSKRSFIEDLLFNKVTLADAGFIKQYGDCLGDIAARDLICAQKFNGLTVLPPLLTDEMIAQYTSALLAGTITSGWTFGAGAALQIPFAMQMAYRFNGIGVTQNVLYENQKLIANQFNSAIGKIQDSLSSTASALGKLQDVVNQNAQALNTLVKQLSSNFGAISSVLNDILSRLDKVEAEVQIDRLITGRLQSLQTYVTQQLIRAAEIRASANLAATKMSECVLGQSKRVDFCGKGYHLMSFPQSAPHGVVFLHVTYVPAQEKNFTTAPAICHDGKAHFPREGVFVSNGTHWFVTQRNFYEPQIITTDNTFVSGNCDVVIGIVNNTVYDPLQPELDSFKEELDKYFKNHTSPDVDLGDISGINASVVNIQKEIDRLNEVAKNLNESLIDLQELGKYEQYIKWPWYIWLGFIAGLIAIVMVTIMLCCMTSCCSCLKGCCSCGSCCKFDEDDSEPVLKGVKLHYT

SEQ ID NO: 11 - protein, 13 aa, Homo sapiens
  REGION 1..13: note = Hinge region of IgG4
ESKYGPPCPPCPA

SEQ ID NO: 12 - protein, 11 aa, Homo sapiens
  REGION 1..11: note = Hinge region of IgG1
DKTHTCPPCPA

SEQ ID NO: 13 - protein, 715 aa, synthetic construct
  REGION 1..715: note = ACE2 18-732 T27A
QSTIEEQAKAFLDKFNHEAEDLFYQSSLASWNYNTNITEENVQNMNNAGDKWSAFLKEQSTLAQMYPLQEIQNLTVKLQLQALQQNGSSVLSEDKSKRLNTILNTMSTIYSTGKVCNPDNPQECLLLEPGLNEIMANSLDYNERLWAWESWRSEVGKQLRPLYEEYVVLKNEMARANHYEDYGDYWRGDYEVNGVDGYDYSRGQLIEDVEHTFEEIKPLYEHLHAYVRAKLMNAYPSYISPIGCLPAHLLGDMWGRFWTNLYSLTVPFGQKPNIDVTDAMVDQAWDAQRIFKEAEKFFVSVGLPNMTQGFWENSMLTDPGNVQKAVCHPTAWDLGKGDFRILMCTKVTMDDFLTAHHEMGHIQYDMAYAAQPFLLRNGANEGFHEAVGEIMSLSAATPKHLKSIGLLSPDFQEDNETEINFLLKQALTIVGTLPFTYMLEKWRWMVFKGEIPKDQWMKKWWEMKREIVGVVEPVPHDETYCDPASLFHVSNDYSFIRYYTRTLYQFQFQEALCQAAKHEGPLHKCDISNSTEAGQKLFNMLRLGKSEPWTLALENVVGAKNMNVRPLLNYFEPLFTWLKDQNKNSFVGWSTDWSPYADQSIKVRISLKSALGDKAYEWNDNEMYLFRSSVAYAMRQYFLKVKNQMILFGEEDVRVANLKPRISFNFFVTAPKNVSDIIPRTEVEKAIRMSRSRINDAFRLNDNSLEFLGIQPTLG

SEQ ID NO: 14 - protein, 715 aa, synthetic construct
  REGION 1..715: note = ACE2 18-732 T92I
QSTIEEQAKTFLDKFNHEAEDLFYQSSLASWNYNTNITEENVQNMNNAGDKWSAFLKEQSTLAQMYPLQEIQNLIVKLQLQALQQNGSSVLSEDKSKRLNTILNTMSTIYSTGKVCNPDNPQECLLLEPGLNEIMANSLDYNERLWAWESWRSEVGKQLRPLYEEYVVLKNEMARANHYEDYGDYWRGDYEVNGVDGYDYSRGQLIEDVEHTFEEIKPLYEHLHAYVRAKLMNAYPSYISPIGCLPAHLLGDMWGRFWTNLYSLTVPFGQKPNIDVTDAMVDQAWDAQRIFKEAEKFFVSVGLPNMTQGFWENSMLTDPGNVQKAVCHPTAWDLGKGDFRILMCTKVTMDDFLTAHHEMGHIQYDMAYAAQPFLLRNGANEGFHEAVGEIMSLSAATPKHLKSIGLLSPDFQEDNETEINFLLKQALTIVGTLPFTYMLEKWRWMVFKGEIPKDQWMKKWWEMKREIVGVVEPVPHDETYCDPASLFHVSNDYSFIRYYTRTLYQFQFQEALCQAAKHEGPLHKCDISNSTEAGQKLFNMLRLGKSEPWTLALENVVGAKNMNVRPLLNYFEPLFTWLKDQNKNSFVGWSTDWSPYADQSIKVRISLKSALGDKAYEWNDNEMYLFRSSVAYAMRQYFLKVKNQMILFGEEDVRVANLKPRISFNFFVTAPKNVSDIIPRTEVEKAIRMSRSRINDAFRLNDNSLEFLGIQPTLG

SEQ ID NO: 15 - protein, 715 aa, synthetic construct
  REGION 1..715: note = ACE2 18-732 Q325P
QSTIEEQAKTFLDKFNHEAEDLFYQSSLASWNYNTNITEENVQNMNNAGDKWSAFLKEQSTLAQMYPLQEIQNLTVKLQLQALQQNGSSVLSEDKSKRLNTILNTMSTIYSTGKVCNPDNPQECLLLEPGLNEIMANSLDYNERLWAWESWRSEVGKQLRPLYEEYVVLKNEMARANHYEDYGDYWRGDYEVNGVDGYDYSRGQLIEDVEHTFEEIKPLYEHLHAYVRAKLMNAYPSYISPIGCLPAHLLGDMWGRFWTNLYSLTVPFGQKPNIDVTDAMVDQAWDAQRIFKEAEKFFVSVGLPNMTPGFWENSMLTDPGNVQKAVCHPTAWDLGKGDFRILMCTKVTMDDFLTAHHEMGHIQYDMAYAAQPFLLRNGANEGFHEAVGEIMSLSAATPKHLKSIGLLSPDFQEDNETEINFLLKQALTIVGTLPFTYMLEKWRWMVFKGEIPKDQWMKKWWEMKREIVGVVEPVPHDETYCDPASLFHVSNDYSFIRYYTRTLYQFQFQEALCQAAKHEGPLHKCDISNSTEAGQKLFNMLRLGKSEPWTLALENVVGAKNMNVRPLLNYFEPLFTWLKDQNKNSFVGWSTDWSPYADQSIKVRISLKSALGDKAYEWNDNEMYLFRSSVAYAMRQYFLKVKNQMILFGEEDVRVANLKPRISFNFFVTAPKNVSDIIPRTEVEKAIRMSRSRINDAFRLNDNSLEFLGIQPTLG

SEQ ID NO: 16 - protein, 715 aa, synthetic construct
  REGION 1..715: note = ACE2 18-732 T27A T92I
QSTIEEQAKAFLDKFNHEAEDLFYQSSLASWNYNTNITEENVQNMNNAGDKWSAFLKEQSTLAQMYPLQEIQNLIVKLQLQALQQNGSSVLSEDKSKRLNTILNTMSTIYSTGKVCNPDNPQECLLLEPGLNEIMANSLDYNERLWAWESWRSEVGKQLRPLYEEYVVLKNEMARANHYEDYGDYWRGDYEVNGVDGYDYSRGQLIEDVEHTFEEIKPLYEHLHAYVRAKLMNAYPSYISPIGCLPAHLLGDMWGRFWTNLYSLTVPFGQKPNIDVTDAMVDQAWDAQRIFKEAEKFFVSVGLPNMTQGFWENSMLTDPGNVQKAVCHPTAWDLGKGDFRILMCTKVTMDDFLTAHHEMGHIQYDMAYAAQPFLLRNGANEGFHEAVGEIMSLSAATPKHLKSIGLLSPDFQEDNETEINFLLKQALTIVGTLPFTYMLEKWRWMVFKGEIPKDQWMKKWWEMKREIVGVVEPVPHDETYCDPASLFHVSNDYSFIRYYTRTLYQFQFQEALCQAAKHEGPLHKCDISNSTEAGQKLFNMLRLGKSEPWTLALENVVGAKNMNVRPLLNYFEPLFTWLKDQNKNSFVGWSTDWSPYADQSIKVRISLKSALGDKAYEWNDNEMYLFRSSVAYAMRQYFLKVKNQMILFGEEDVRVANLKPRISFNFFVTAPKNVSDIIPRTEVEKAIRMSRSRINDAFRLNDNSLEFLGIQPTLG

SEQ ID NO: 17 - protein, 715 aa, synthetic construct
  REGION 1..715: note = ACE2 18-732 T27A Q325P
QSTIEEQAKAFLDKFNHEAEDLFYQSSLASWNYNTNITEENVQNMNNAGDKWSAFLKEQSTLAQMYPLQEIQNLTVKLQLQALQQNGSSVLSEDKSKRLNTILNTMSTIYSTGKVCNPDNPQECLLLEPGLNEIMANSLDYNERLWAWESWRSEVGKQLRPLYEEYVVLKNEMARANHYEDYGDYWRGDYEVNGVDGYDYSRGQLIEDVEHTFEEIKPLYEHLHAYVRAKLMNAYPSYISPIGCLPAHLLGDMWGRFWTNLYSLTVPFGQKPNIDVTDAMVDQAWDAQRIFKEAEKFFVSVGLPNMTPGFWENSMLTDPGNVQKAVCHPTAWDLGKGDFRILMCTKVTMDDFLTAHHEMGHIQYDMAYAAQPFLLRNGANEGFHEAVGEIMSLSAATPKHLKSIGLLSPDFQEDNETEINFLLKQALTIVGTLPFTYMLEKWRWMVFKGEIPKDQWMKKWWEMKREIVGVVEPVPHDETYCDPASLFHVSNDYSFIRYYTRTLYQFQFQEALCQAAKHEGPLHKCDISNSTEAGQKLFNMLRLGKSEPWTLALENVVGAKNMNVRPLLNYFEPLFTWLKDQNKNSFVGWSTDWSPYADQSIKVRISLKSALGDKAYEWNDNEMYLFRSSVAYAMRQYFLKVKNQMILFGEEDVRVANLKPRISFNFFVTAPKNVSDIIPRTEVEKAIRMSRSRINDAFRLNDNSLEFLGIQPTLG

SEQ ID NO: 18 - protein, 715 aa, synthetic construct
  REGION 1..715: note = ACE2 18-732 T92I Q325P
QSTIEEQAKTFLDKFNHEAEDLFYQSSLASWNYNTNITEENVQNMNNAGDKWSAFLKEQSTLAQMYPLQEIQNLIVKLQLQALQQNGSSVLSEDKSKRLNTILNTMSTIYSTGKVCNPDNPQECLLLEPGLNEIMANSLDYNERLWAWESWRSEVGKQLRPLYEEYVVLKNEMARANHYEDYGDYWRGDYEVNGVDGYDYSRGQLIEDVEHTFEEIKPLYEHLHAYVRAKLMNAYPSYISPIGCLPAHLLGDMWGRFWTNLYSLTVPFGQKPNIDVTDAMVDQAWDAQRIFKEAEKFFVSVGLPNMTPGFWENSMLTDPGNVQKAVCHPTAWDLGKGDFRILMCTKVTMDDFLTAHHEMGHIQYDMAYAAQPFLLRNGANEGFHEAVGEIMSLSAATPKHLKSIGLLSPDFQEDNETEINFLLKQALTIVGTLPFTYMLEKWRWMVFKGEIPKDQWMKKWWEMKREIVGVVEPVPHDETYCDPASLFHVSNDYSFIRYYTRTLYQFQFQEALCQAAKHEGPLHKCDISNSTEAGQKLFNMLRLGKSEPWTLALENVVGAKNMNVRPLLNYFEPLFTWLKDQNKNSFVGWSTDWSPYADQSIKVRISLKSALGDKAYEWNDNEMYLFRSSVAYAMRQYFLKVKNQMILFGEEDVRVANLKPRISFNFFVTAPKNVSDIIPRTEVEKAIRMSRSRINDAFRLNDNSLEFLGIQPTLG

SEQ ID NO: 19 - protein, 715 aa, synthetic construct
  REGION 1..715: note = ACE2 18-732 T27A T92I Q325P
QSTIEEQAKAFLDKFNHEAEDLFYQSSLASWNYNTNITEENVQNMNNAGDKWSAFLKEQSTLAQMYPLQEIQNLIVKLQLQALQQNGSSVLSEDKSKRLNTILNTMSTIYSTGKVCNPDNPQECLLLEPGLNEIMANSLDYNERLWAWESWRSEVGKQLRPLYEEYVVLKNEMARANHYEDYGDYWRGDYEVNGVDGYDYSRGQLIEDVEHTFEEIKPLYEHLHAYVRAKLMNAYPSYISPIGCLPAHLLGDMWGRFWTNLYSLTVPFGQKPNIDVTDAMVDQAWDAQRIFKEAEKFFVSVGLPNMTPGFWENSMLTDPGNVQKAVCHPTAWDLGKGDFRILMCTKVTMDDFLTAHHEMGHIQYDMAYAAQPFLLRNGANEGFHEAVGEIMSLSAATPKHLKSIGLLSPDFQEDNETEINFLLKQALTIVGTLPFTYMLEKWRWMVFKGEIPKDQWMKKWWEMKREIVGVVEPVPHDETYCDPASLFHVSNDYSFIRYYTRTLYQFQFQEALCQAAKHEGPLHKCDISNSTEAGQKLFNMLRLGKSEPWTLALENVVGAKNMNVRPLLNYFEPLFTWLKDQNKNSFVGWSTDWSPYADQSIKVRISLKSALGDKAYEWNDNEMYLFRSSVAYAMRQYFLKVKNQMILFGEEDVRVANLKPRISFNFFVTAPKNVSDIIPRTEVEKAIRMSRSRINDAFRLNDNSLEFLGIQPTLG

SEQ ID NO: 20 - protein, 715 aa, synthetic construct
  REGION 1..715: note = ACE2 18-732 T27A S645C
QSTIEEQAKAFLDKFNHEAEDLFYQSSLASWNYNTNITEENVQNMNNAGDKWSAFLKEQSTLAQMYPLQEIQNLTVKLQLQALQQNGSSVLSEDKSKRLNTILNTMSTIYSTGKVCNPDNPQECLLLEPGLNEIMANSLDYNERLWAWESWRSEVGKQLRPLYEEYVVLKNEMARANHYEDYGDYWRGDYEVNGVDGYDYSRGQLIEDVEHTFEEIKPLYEHLHAYVRAKLMNAYPSYISPIGCLPAHLLGDMWGRFWTNLYSLTVPFGQKPNIDVTDAMVDQAWDAQRIFKEAEKFFVSVGLPNMTQGFWENSMLTDPGNVQKAVCHPTAWDLGKGDFRILMCTKVTMDDFLTAHHEMGHIQYDMAYAAQPFLLRNGANEGFHEAVGEIMSLSAATPKHLKSIGLLSPDFQEDNETEINFLLKQALTIVGTLPFTYMLEKWRWMVFKGEIPKDQWMKKWWEMKREIVGVVEPVPHDETYCDPASLFHVSNDYSFIRYYTRTLYQFQFQEALCQAAKHEGPLHKCDISNSTEAGQKLFNMLRLGKSEPWTLALENVVGAKNMNVRPLLNYFEPLFTWLKDQNKNSFVGWSTDWSPYADQSIKVRISLKSALGDKAYEWNDNEMYLFRCSVAYAMRQYFLKVKNQMILFGEEDVRVANLKPRISFNFFVTAPKNVSDIIPRTEVEKAIRMSRSRINDAFRLNDNSLEFLGIQPTLG

SEQ ID NO: 21 - protein, 715 aa, synthetic construct
  REGION 1..715: note = ACE2 18-732 T92I S645C
QSTIEEQAKTFLDKFNHEAEDLFYQSSLASWNYNTNITEENVQNMNNAGDKWSAFLKEQSTLAQMYPLQEIQNLIVKLQLQALQQNGSSVLSEDKSKRLNTILNTMSTIYSTGKVCNPDNPQECLLLEPGLNEIMANSLDYNERLWAWESWRSEVGKQLRPLYEEYVVLKNEMARANHYEDYGDYWRGDYEVNGVDGYDYSRGQLIEDVEHTFEEIKPLYEHLHAYVRAKLMNAYPSYISPIGCLPAHLLGDMWGRFWTNLYSLTVPFGQKPNIDVTDAMVDQAWDAQRIFKEAEKFFVSVGLPNMTQGFWENSMLTDPGNVQKAVCHPTAWDLGKGDFRILMCTKVTMDDFLTAHHEMGHIQYDMAYAAQPFLLRNGANEGFHEAVGEIMSLSAATPKHLKSIGLLSPDFQEDNETEINFLLKQALTIVGTLPFTYMLEKWRWMVFKGEIPKDQWMKKWWEMKREIVGVVEPVPHDETYCDPASLFHVSNDYSFIRYYTRTLYQFQFQEALCQAAKHEGPLHKCDISNSTEAGQKLFNMLRLGKSEPWTLALENVVGAKNMNVRPLLNYFEPLFTWLKDQNKNSFVGWSTDWSPYADQSIKVRISLKSALGDKAYEWNDNEMYLFRCSVAYAMRQYFLKVKNQMILFGEEDVRVANLKPRISFNFFVTAPKNVSDIIPRTEVEKAIRMSRSRINDAFRLNDNSLEFLGIQPTLG

SEQ ID NO: 22 - protein, 715 aa, synthetic construct
  REGION 1..715: note = ACE2 18-732 Q325P S645C
QSTIEEQAKTFLDKFNHEAEDLFYQSSLASWNYNTNITEENVQNMNNAGDKWSAFLKEQSTLAQMYPLQEIQNLTVKLQLQALQQNGSSVLSEDKSKRLNTILNTMSTIYSTGKVCNPDNPQECLLLEPGLNEIMANSLDYNERLWAWESWRSEVGKQLRPLYEEYVVLKNEMARANHYEDYGDYWRGDYEVNGVDGYDYSRGQLIEDVEHTFEEIKPLYEHLHAYVRAKLMNAYPSYISPIGCLPAHLLGDMWGRFWTNLYSLTVPFGQKPNIDVTDAMVDQAWDAQRIFKEAEKFFVSVGLPNMTPGFWENSMLTDPGNVQKAVCHPTAWDLGKGDFRILMCTKVTMDDFLTAHHEMGHIQYDMAYAAQPFLLRNGANEGFHEAVGEIMSLSAATPKHLKSIGLLSPDFQEDNETEINFLLKQALTIVGTLPFTYMLEKWRWMVFKGEIPKDQWMKKWWEMKREIVGVVEPVPHDETYCDPASLFHVSNDYSFIRYYTRTLYQFQFQEALCQAAKHEGPLHKCDISNSTEAGQKLFNMLRLGKSEPWTLALENVVGAKNMNVRPLLNYFEPLFTWLKDQNKNSFVGWSTDWSPYADQSIKVRISLKSALGDKAYEWNDNEMYLFRCSVAYAMRQYFLKVKNQMILFGEEDVRVANLKPRISFNFFVTAPKNVSDIIPRTEVEKAIRMSRSRINDAFRLNDNSLEFLGIQPTLG

SEQ ID NO: 23 - protein, 715 aa, synthetic construct
  REGION 1..715: note = ACE2 18-732 T27A T92I S645C
QSTIEEQAKAFLDKFNHEAEDLFYQSSLASWNYNTNITEENVQNMNNAGDKWSAFLKEQSTLAQMYPLQEIQNLIVKLQLQALQQNGSSVLSEDKSKRLNTILNTMSTIYSTGKVCNPDNPQECLLLEPGLNEIMANSLDYNERLWAWESWRSEVGKQLRPLYEEYVVLKNEMARANHYEDYGDYWRGDYEVNGVDGYDYSRGQLIEDVEHTFEEIKPLYEHLHAYVRAKLMNAYPSYISPIGCLPAHLLGDMWGRFWTNLYSLTVPFGQKPNIDVTDAMVDQAWDAQRIFKEAEKFFVSVGLPNMTQGFWENSMLTDPGNVQKAVCHPTAWDLGKGDFRILMCTKVTMDDFLTAHHEMGHIQYDMAYAAQPFLLRNGANEGFHEAVGEIMSLSAATPKHLKSIGLLSPDFQEDNETEINFLLKQALTIVGTLPFTYMLEKWRWMVFKGEIPKDQWMKKWWEMKREIVGVVEPVPHDETYCDPASLFHVSNDYSFIRYYTRTLYQFQFQEALCQAAKHEGPLHKCDISNSTEAGQKLFNMLRLGKSEPWTLALENVVGAKNMNVRPLLNYFEPLFTWLKDQNKNSFVGWSTDWSPYADQSIKVRISLKSALGDKAYEWNDNEMYLFRCSVAYAMRQYFLKVKNQMILFGEEDVRVANLKPRISFNFFVTAPKNVSDIIPRTEVEKAIRMSRSRINDAFRLNDNSLEFLGIQPTLG

SEQ ID NO: 24 - protein, 715 aa, synthetic construct
  REGION 1..715: note = ACE2 18-732 T27A Q325P S645C
QSTIEEQAKAFLDKFNHEAEDLFYQSSLASWNYNTNITEENVQNMNNAGDKWSAFLKEQSTLAQMYPLQEIQNLTVKLQLQALQQNGSSVLSEDKSKRLNTILNTMSTIYSTGKVCNPDNPQECLLLEPGLNEIMANSLDYNERLWAWESWRSEVGKQLRPLYEEYVVLKNEMARANHYEDYGDYWRGDYEVNGVDGYDYSRGQLIEDVEHTFEEIKPLYEHLHAYVRAKLMNAYPSYISPIGCLPAHLLGDMWGRFWTNLYSLTVPFGQKPNIDVTDAMVDQAWDAQRIFKEAEKFFVSVGLPNMTPGFWENSMLTDPGNVQKAVCHPTAWDLGKGDFRILMCTKVTMDDFLTAHHEMGHIQYDMAYAAQPFLLRNGANEGFHEAVGEIMSLSAATPKHLKSIGLLSPDFQEDNETEINFLLKQALTIVGTLPFTYMLEKWRWMVFKGEIPKDQWMKKWWEMKREIVGVVEPVPHDETYCDPASLFHVSNDYSFIRYYTRTLYQFQFQEALCQAAKHEGPLHKCDISNSTEAGQKLFNMLRLGKSEPWTLALENVVGAKNMNVRPLLNYFEPLFTWLKDQNKNSFVGWSTDWSPYADQSIKVRISLKSALGDKAYEWNDNEMYLFRCSVAYAMRQYFLKVKNQMILFGEEDVRVANLKPRISFNFFVTAPKNVSDIIPRTEVEKAIRMSRSRINDAFRLNDNSLEFLGIQPTLG

SEQ ID NO: 25 - protein, 715 aa, synthetic construct
  REGION 1..715: note = ACE2 18-732 T92I Q325P S645C
QSTIEEQAKTFLDKFNHEAEDLFYQSSLASWNYNTNITEENVQNMNNAGDKWSAFLKEQSTLAQMYPLQEIQNLIVKLQLQALQQNGSSVLSEDKSKRLNTILNTMSTIYSTGKVCNPDNPQECLLLEPGLNEIMANSLDYNERLWAWESWRSEVGKQLRPLYEEYVVLKNEMARANHYEDYGDYWRGDYEVNGVDGYDYSRGQLIEDVEHTFEEIKPLYEHLHAYVRAKLMNAYPSYISPIGCLPAHLLGDMWGRFWTNLYSLTVPFGQKPNIDVTDAMVDQAWDAQRIFKEAEKFFVSVGLPNMTPGFWENSMLTDPGNVQKAVCHPTAWDLGKGDFRILMCTKVTMDDFLTAHHEMGHIQYDMAYAAQPFLLRNGANEGFHEAVGEIMSLSAATPKHLKSIGLLSPDFQEDNETEINFLLKQALTIVGTLPFTYMLEKWRWMVFKGEIPKDQWMKKWWEMKREIVGVVEPVPHDETYCDPASLFHVSNDYSFIRYYTRTLYQFQFQEALCQAAKHEGPLHKCDISNSTEAGQKLFNMLRLGKSEPWTLALENVVGAKNMNVRPLLNYFEPLFTWLKDQNKNSFVGWSTDWSPYADQSIKVRISLKSALGDKAYEWNDNEMYLFRCSVAYAMRQYFLKVKNQMILFGEEDVRVANLKPRISFNFFVTAPKNVSDIIPRTEVEKAIRMSRSRINDAFRLNDNSLEFLGIQPTLG

SEQ ID NO: 26 - protein, 715 aa, synthetic construct
  REGION 1..715: note = ACE2 18-732 T27A T92I Q325P S645C
QSTIEEQAKAFLDKFNHEAEDLFYQSSLASWNYNTNITEENVQNMNNAGDKWSAFLKEQSTLAQMYPLQEIQNLIVKLQLQALQQNGSSVLSEDKSKRLNTILNTMSTIYSTGKVCNPDNPQECLLLEPGLNEIMANSLDYNERLWAWESWRSEVGKQLRPLYEEYVVLKNEMARANHYEDYGDYWRGDYEVNGVDGYDYSRGQLIEDVEHTFEEIKPLYEHLHAYVRAKLMNAYPSYISPIGCLPAHLLGDMWGRFWTNLYSLTVPFGQKPNIDVTDAMVDQAWDAQRIFKEAEKFFVSVGLPNMTPGFWENSMLTDPGNVQKAVCHPTAWDLGKGDFRILMCTKVTMDDFLTAHHEMGHIQYDMAYAAQPFLLRNGANEGFHEAVGEIMSLSAATPKHLKSIGLLSPDFQEDNETEINFLLKQALTIVGTLPFTYMLEKWRWMVFKGEIPKDQWMKKWWEMKREIVGVVEPVPHDETYCDPASLFHVSNDYSFIRYYTRTLYQFQFQEALCQAAKHEGPLHKCDISNSTEAGQKLFNMLRLGKSEPWTLALENVVGAKNMNVRPLLNYFEPLFTWLKDQNKNSFVGWSTDWSPYADQSIKVRISLKSALGDKAYEWNDNEMYLFRCSVAYAMRQYFLKVKNQMILFGEEDVRVANLKPRISFNFFVTAPKNVSDIIPRTEVEKAIRMSRSRINDAFRLNDNSLEFLGIQPTLG

SEQ ID NO: 27 - protein, 944 aa, synthetic construct
  REGION 1..944: note = ACE2 18-732 T27A IgG4 YTE
QSTIEEQAKAFLDKFNHEAEDLFYQSSLASWNYNTNITEENVQNMNNAGDKWSAFLKEQSTLAQMYPLQEIQNLTVKLQLQALQQNGSSVLSEDKSKRLNTILNTMSTIYSTGKVCNPDNPQECLLLEPGLNEIMANSLDYNERLWAWESWRSEVGKQLRPLYEEYVVLKNEMARANHYEDYGDYWRGDYEVNGVDGYDYSRGQLIEDVEHTFEEIKPLYEHLHAYVRAKLMNAYPSYISPIGCLPAHLLGDMWGRFWTNLYSLTVPFGQKPNIDVTDAMVDQAWDAQRIFKEAEKFFVSVGLPNMTQGFWENSMLTDPGNVQKAVCHPTAWDLGKGDFRILMCTKVTMDDFLTAHHEMGHIQYDMAYAAQPFLLRNGANEGFHEAVGEIMSLSAATPKHLKSIGLLSPDFQEDNETEINFLLKQALTIVGTLPFTYMLEKWRWMVFKGEIPKDQWMKKWWEMKREIVGVVEPVPHDETYCDPASLFHVSNDYSFIRYYTRTLYQFQFQEALCQAAKHEGPLHKCDISNSTEAGQKLFNMLRLGKSEPWTLALENVVGAKNMNVRPLLNYFEPLFTWLKDQNKNSFVGWSTDWSPYADQSIKVRISLKSALGDKAYEWNDNEMYLFRSSVAYAMRQYFLKVKNQMILFGEEDVRVANLKPRISFNFFVTAPKNVSDIIPRTEVEKAIRMSRSRINDAFRLNDNSLEFLGIQPTLGESKYGPPCPPCPAPEFLGGPSVFLFPPKPKDTLYITREPEVTCVVVDVSQEDPEVQFNWYVDGVEVHNAKTKPREEQFNSTYRVVSVLTVLHQDWLNGKEYKCKVSNKGLPSSIEKTISKAKGQPREPQVYTLPPSQEEMTKNQVSLTCLVKGFYPSDIAVEWESNGQPENNYKTTPPVLDSDGSFFLYSRLTVDKSRWQEGNVFSCSVMHEALHNHYTQKSLSLSLGK

SEQ ID NO: 28 - protein, 942 aa, synthetic construct
  REGION 1..942: note = ACE2 18-732 T27A IgG1 YTE
QSTIEEQAKAFLDKFNHEAEDLFYQSSLASWNYNTNITEENVQNMNNAGDKWSAFLKEQSTLAQMYPLQEIQNLTVKLQLQALQQNGSSVLSEDKSKRLNTILNTMSTIYSTGKVCNPDNPQECLLLEPGLNEIMANSLDYNERLWAWESWRSEVGKQLRPLYEEYVVLKNEMARANHYEDYGDYWRGDYEVNGVDGYDYSRGQLIEDVEHTFEEIKPLYEHLHAYVRAKLMNAYPSYISPIGCLPAHLLGDMWGRFWTNLYSLTVPFGQKPNIDVTDAMVDQAWDAQRIFKEAEKFFVSVGLPNMTQGFWENSMLTDPGNVQKAVCHPTAWDLGKGDFRILMCTKVTMDDFLTAHHEMGHIQYDMAYAAQPFLLRNGANEGFHEAVGEIMSLSAATPKHLKSIGLLSPDFQEDNETEINFLLKQALTIVGTLPFTYMLEKWRWMVFKGEIPKDQWMKKWWEMKREIVGVVEPVPHDETYCDPASLFHVSNDYSFIRYYTRTLYQFQFQEALCQAAKHEGPLHKCDISNSTEAGQKLFNMLRLGKSEPWTLALENVVGAKNMNVRPLLNYFEPLFTWLKDQNKNSFVGWSTDWSPYADQSIKVRISLKSALGDKAYEWNDNEMYLFRSSVAYAMRQYFLKVKNQMILFGEEDVRVANLKPRISFNFFVTAPKNVSDIIPRTEVEKAIRMSRSRINDAFRLNDNSLEFLGIQPTLGDKTHTCPPCPAPELLGGPSVFLFPPKPKDTLYITREPEVTCVVVDVSHEDPEVKFNWYVDGVEVHNAKTKPREEQYNSTYRVVSVLTVLHQDWLNGKEYKCKVSNKALPAPIEKTISKAKGQPREPQVYTLPPSRDELTKNQVSLTCLVKGFYPSDIAVEWESNGQPENNYKTTPPVLDSDGSFFLYSKLTVDKSRWQQGNVFSCSVMHEALHNHYTQKSLSLSPGK

SEQ ID NO: 29 - protein, 944 aa, synthetic construct
  REGION 1..944: note = ACE2 18-732 T27A IgG4 T256D T307Q
QSTIEEQAKAFLDKFNHEAEDLFYQSSLASWNYNTNITEENVQNMNNAGDKWSAFLKEQSTLAQMYPLQEIQNLTVKLQLQALQQNGSSVLSEDKSKRLNTILNTMSTIYSTGKVCNPDNPQECLLLEPGLNEIMANSLDYNERLWAWESWRSEVGKQLRPLYEEYVVLKNEMARANHYEDYGDYWRGDYEVNGVDGYDYSRGQLIEDVEHTFEEIKPLYEHLHAYVRAKLMNAYPSYISPIGCLPAHLLGDMWGRFWTNLYSLTVPFGQKPNIDVTDAMVDQAWDAQRIFKEAEKFFVSVGLPNMTQGFWENSMLTDPGNVQKAVCHPTAWDLGKGDFRILMCTKVTMDDFLTAHHEMGHIQYDMAYAAQPFLLRNGANEGFHEAVGEIMSLSAATPKHLKSIGLLSPDFQEDNETEINFLLKQALTIVGTLPFTYMLEKWRWMVFKGEIPKDQWMKKWWEMKREIVGVVEPVPHDETYCDPASLFHVSNDYSFIRYYTRTLYQFQFQEALCQAAKHEGPLHKCDISNSTEAGQKLFNMLRLGKSEPWTLALENVVGAKNMNVRPLLNYFEPLFTWLKDQNKNSFVGWSTDWSPYADQSIKVRISLKSALGDKAYEWNDNEMYLFRSSVAYAMRQYFLKVKNQMILFGEEDVRVANLKPRISFNFFVTAPKNVSDIIPRTEVEKAIRMSRSRINDAFRLNDNSLEFLGIQPTLGESKYGPPCPPCPAPEFLGGPSVFLFPPKPKDTLMISRDPEVTCVVVDVSQEDPEVQFNWYVDGVEVHNAKTKPREEQFNSTYRVVSVLQVLHQDWLNGKEYKCKVSNKGLPSSIEKTISKAKGQPREPQVYTLPPSQEEMTKNQVSLTCLVKGFYPSDIAVEWESNGQPENNYKTTPPVLDSDGSFFLYSRLTVDKSRWQEGNVFSCSVMHEALHNHYTQKSLSLSLGK

SEQ ID NO: 30 - protein, 942 aa, synthetic construct
  REGION 1..942: note = ACE2 18-732 T27A IgG1 T256D T307Q
QSTIEEQAKAFLDKFNHEAEDLFYQSSLASWNYNTNITEENVQNMNNAGDKWSAFLKEQSTLAQMYPLQEIQNLTVKLQLQALQQNGSSVLSEDKSKRLNTILNTMSTIYSTGKVCNPDNPQECLLLEPGLNEIMANSLDYNERLWAWESWRSEVGKQLRPLYEEYVVLKNEMARANHYEDYGDYWRGDYEVNGVDGYDYSRGQLIEDVEHTFEEIKPLYEHLHAYVRAKLMNAYPSYISPIGCLPAHLLGDMWGRFWTNLYSLTVPFGQKPNIDVTDAMVDQAWDAQRIFKEAEKFFVSVGLPNMTQGFWENSMLTDPGNVQKAVCHPTAWDLGKGDFRILMCTKVTMDDFLTAHHEMGHIQYDMAYAAQPFLLRNGANEGFHEAVGEIMSLSAATPKHLKSIGLLSPDFQEDNETEINFLLKQALTIVGTLPFTYMLEKWRWMVFKGEIPKDQWMKKWWEMKREIVGVVEPVPHDETYCDPASLFHVSNDYSFIRYYTRTLYQFQFQEALCQAAKHEGPLHKCDISNSTEAGQKLFNMLRLGKSEPWTLALENVVGAKNMNVRPLLNYFEPLFTWLKDQNKNSFVGWSTDWSPYADQSIKVRISLKSALGDKAYEWNDNEMYLFRSSVAYAMRQYFLKVKNQMILFGEEDVRVANLKPRISFNFFVTAPKNVSDIIPRTEVEKAIRMSRSRINDAFRLNDNSLEFLGIQPTLGDKTHTCPPCPAPELLGGPSVFLFPPKPKDTLMISRDPEVTCVVVDVSHEDPEVKFNWYVDGVEVHNAKTKPREEQYNSTYRVVSVLQVLHQDWLNGKEYKCKVSNKALPAPIEKTISKAKGQPREPQVYTLPPSRDELTKNQVSLTCLVKGFYPSDIAVEWESNGQPENNYKTTPPVLDSDGSFFLYSKLTVDKSRWQQGNVFSCSVMHEALHNHYTQKSLSLSPGK

SEQ ID NO: 31 - protein, 944 aa, synthetic construct
  REGION 1..943: note = ACE2 18-732 T92I IgG4 YTE
QSTIEEQAKTFLDKFNHEAEDLFYQSSLASWNYNTNITEENVQNMNNAGDKWSAFLKEQSTLAQMYPLQEIQNLIVKLQLQALQQNGSSVLSEDKSKRLNTILNTMSTIYSTGKVCNPDNPQECLLLEPGLNEIMANSLDYNERLWAWESWRSEVGKQLRPLYEEYVVLKNEMARANHYEDYGDYWRGDYEVNGVDGYDYSRGQLIEDVEHTFEEIKPLYEHLHAYVRAKLMNAYPSYISPIGCLPAHLLGDMWGRFWTNLYSLTVPFGQKPNIDVTDAMVDQAWDAQRIFKEAEKFFVSVGLPNMTQGFWENSMLTDPGNVQKAVCHPTAWDLGKGDFRILMCTKVTMDDFLTAHHEMGHIQYDMAYAAQPFLLRNGANEGFHEAVGEIMSLSAATPKHLKSIGLLSPDFQEDNETEINFLLKQALTIVGTLPFTYMLEKWRWMVFKGEIPKDQWMKKWWEMKREIVGVVEPVPHDETYCDPASLFHVSNDYSFIRYYTRTLYQFQFQEALCQAAKHEGPLHKCDISNSTEAGQKLFNMLRLGKSEPWTLALENVVGAKNMNVRPLLNYFEPLFTWLKDQNKNSFVGWSTDWSPYADQSIKVRISLKSALGDKAYEWNDNEMYLFRSSVAYAMRQYFLKVKNQMILFGEEDVRVANLKPRISFNFFVTAPKNVSDIIPRTEVEKAIRMSRSRINDAFRLNDNSLEFLGIQPTLGESKYGPPCPPCPAPEFLGGPSVFLFPPKPKDTLYITREPEVTCVVVDVSQEDPEVQFNWYVDGVEVHNAKTKPREEQFNSTYRVVSVLTVLHQDWLNGKEYKCKVSNKGLPSSIEKTISKAKGQPREPQVYTLPPSQEEMTKNQVSLTCLVKGFYPSDIAVEWESNGQPENNYKTTPPVLDSDGSFFLYSRLTVDKSRWQEGNVFSCSVMHEALHNHYTQKSLSLSLGK

SEQ ID NO: 32 - protein, 942 aa, synthetic construct
  REGION 1..942: note = ACE2 18-732 T92I IgG1 YTE
QSTIEEQAKTFLDKFNHEAEDLFYQSSLASWNYNTNITEENVQNMNNAGDKWSAFLKEQSTLAQMYPLQEIQNLIVKLQLQALQQNGSSVLSEDKSKRLNTILNTMSTIYSTGKVCNPDNPQECLLLEPGLNEIMANSLDYNERLWAWESWRSEVGKQLRPLYEEYVVLKNEMARANHYEDYGDYWRGDYEVNGVDGYDYSRGQLIEDVEHTFEEIKPLYEHLHAYVRAKLMNAYPSYISPIGCLPAHLLGDMWGRFWTNLYSLTVPFGQKPNIDVTDAMVDQAWDAQRIFKEAEKFFVSVGLPNMTQGFWENSMLTDPGNVQKAVCHPTAWDLGKGDFRILMCTKVTMDDFLTAHHEMGHIQYDMAYAAQPFLLRNGANEGFHEAVGEIMSLSAATPKHLKSIGLLSPDFQEDNETEINFLLKQALTIVGTLPFTYMLEKWRWMVFKGEIPKDQWMKKWWEMKREIVGVVEPVPHDETYCDPASLFHVSNDYSFIRYYTRTLYQFQFQEALCQAAKHEGPLHKCDISNSTEAGQKLFNMLRLGKSEPWTLALENVVGAKNMNVRPLLNYFEPLFTWLKDQNKNSFVGWSTDWSPYADQSIKVRISLKSALGDKAYEWNDNEMYLFRSSVAYAMRQYFLKVKNQMILFGEEDVRVANLKPRISFNFFVTAPKNVSDIIPRTEVEKAIRMSRSRINDAFRLNDNSLEFLGIQPTLGDKTHTCPPCPAPELLGGPSVFLFPPKPKDTLYITREPEVTCVVVDVSHEDPEVKFNWYVDGVEVHNAKTKPREEQYNSTYRVVSVLTVLHQDWLNGKEYKCKVSNKALPAPIEKTISKAKGQPREPQVYTLPPSRDELTKNQVSLTCLVKGFYPSDIAVEWESNGQPENNYKTTPPVLDSDGSFFLYSKLTVDKSRWQQGNVFSCSVMHEALHNHYTQKSLSLSPGK

SEQ ID NO: 33 - protein, 944 aa, synthetic construct
  REGION 1..944: note = ACE2 18-732 T92I IgG4 T256D T307Q
QSTIEEQAKTFLDKFNHEAEDLFYQSSLASWNYNTNITEENVQNMNNAGDKWSAFLKEQSTLAQMYPLQEIQNLIVKLQLQALQQNGSSVLSEDKSKRLNTILNTMSTIYSTGKVCNPDNPQECLLLEPGLNEIMANSLDYNERLWAWESWRSEVGKQLRPLYEEYVVLKNEMARANHYEDYGDYWRGDYEVNGVDGYDYSRGQLIEDVEHTFEEIKPLYEHLHAYVRAKLMNAYPSYISPIGCLPAHLLGDMWGRFWTNLYSLTVPFGQKPNIDVTDAMVDQAWDAQRIFKEAEKFFVSVGLPNMTQGFWENSMLTDPGNVQKAVCHPTAWDLGKGDFRILMCTKVTMDDFLTAHHEMGHIQYDMAYAAQPFLLRNGANEGFHEAVGEIMSLSAATPKHLKSIGLLSPDFQEDNETEINFLLKQALTIVGTLPFTYMLEKWRWMVFKGEIPKDQWMKKWWEMKREIVGVVEPVPHDETYCDPASLFHVSNDYSFIRYYTRTLYQFQFQEALCQAAKHEGPLHKCDISNSTEAGQKLFNMLRLGKSEPWTLALENVVGAKNMNVRPLLNYFEPLFTWLKDQNKNSFVGWSTDWSPYADQSIKVRISLKSALGDKAYEWNDNEMYLFRSSVAYAMRQYFLKVKNQMILFGEEDVRVANLKPRISFNFFVTAPKNVSDIIPRTEVEKAIRMSRSRINDAFRLNDNSLEFLGIQPTLGESKYGPPCPPCPAPEFLGGPSVFLFPPKPKDTLMISRDPEVTCVVVDVSQEDPEVQFNWYVDGVEVHNAKTKPREEQFNSTYRVVSVLQVLHQDWLNGKEYKCKVSNKGLPSSIEKTISKAKGQPREPQVYTLPPSQEEMTKNQVSLTCLVKGFYPSDIAVEWESNGQPENNYKTTPPVLDSDGSFFLYSRLTVDKSRWQEGNVFSCSVMHEALHNHYTQKSLSLSLGK

SEQ ID NO: 34 - protein, 942 aa, synthetic construct
  REGION 1..942: note = ACE2 18-732 T92I IgG1 T256D T307Q
QSTIEEQAKTFLDKFNHEAEDLFYQSSLASWNYNTNITEENVQNMNNAGDKWSAFLKEQSTLAQMYPLQEIQNLIVKLQLQALQQNGSSVLSEDKSKRLNTILNTMSTIYSTGKVCNPDNPQECLLLEPGLNEIMANSLDYNERLWAWESWRSEVGKQLRPLYEEYVVLKNEMARANHYEDYGDYWRGDYEVNGVDGYDYSRGQLIEDVEHTFEEIKPLYEHLHAYVRAKLMNAYPSYISPIGCLPAHLLGDMWGRFWTNLYSLTVPFGQKPNIDVTDAMVDQAWDAQRIFKEAEKFFVSVGLPNMTQGFWENSMLTDPGNVQKAVCHPTAWDLGKGDFRILMCTKVTMDDFLTAHHEMGHIQYDMAYAAQPFLLRNGANEGFHEAVGEIMSLSAATPKHLKSIGLLSPDFQEDNETEINFLLKQALTIVGTLPFTYMLEKWRWMVFKGEIPKDQWMKKWWEMKREIVGVVEPVPHDETYCDPASLFHVSNDYSFIRYYTRTLYQFQFQEALCQAAKHEGPLHKCDISNSTEAGQKLFNMLRLGKSEPWTLALENVVGAKNMNVRPLLNYFEPLFTWLKDQNKNSFVGWSTDWSPYADQSIKVRISLKSALGDKAYEWNDNEMYLFRSSVAYAMRQYFLKVKNQMILFGEEDVRVANLKPRISFNFFVTAPKNVSDIIPRTEVEKAIRMSRSRINDAFRLNDNSLEFLGIQPTLGDKTHTCPPCPAPELLGGPSVFLFPPKPKDTLMISRDPEVTCVVVDVSHEDPEVKFNWYVDGVEVHNAKTKPREEQYNSTYRVVSVLQVLHQDWLNGKEYKCKVSNKALPAPIEKTISKAKGQPREPQVYTLPPSRDELTKNQVSLTCLVKGFYPSDIAVEWESNGQPENNYKTTPPVLDSDGSFFLYSKLTVDKSRWQQGNVFSCSVMHEALHNHYTQKSLSLSPGK

SEQ ID NO: 35 - protein, 944 aa, synthetic construct
  REGION 1..715: note = ACE2 18-732 Q325P IgG4 YTE
QSTIEEQAKTFLDKFNHEAEDLFYQSSLASWNYNTNITEENVQNMNNAGDKWSAFLKEQSTLAQMYPLQEIQNLTVKLQLQALQQNGSSVLSEDKSKRLNTILNTMSTIYSTGKVCNPDNPQECLLLEPGLNEIMANSLDYNERLWAWESWRSEVGKQLRPLYEEYVVLKNEMARANHYEDYGDYWRGDYEVNGVDGYDYSRGQLIEDVEHTFEEIKPLYEHLHAYVRAKLMNAYPSYISPIGCLPAHLLGDMWGRFWTNLYSLTVPFGQKPNIDVTDAMVDQAWDAQRIFKEAEKFFVSVGLPNMTPGFWENSMLTDPGNVQKAVCHPTAWDLGKGDFRILMCTKVTMDDFLTAHHEMGHIQYDMAYAAQPFLLRNGANEGFHEAVGEIMSLSAATPKHLKSIGLLSPDFQEDNETEINFLLKQALTIVGTLPFTYMLEKWRWMVFKGEIPKDQWMKKWWEMKREIVGVVEPVPHDETYCDPASLFHVSNDYSFIRYYTRTLYQFQFQEALCQAAKHEGPLHKCDISNSTEAGQKLFNMLRLGKSEPWTLALENVVGAKNMNVRPLLNYFEPLFTWLKDQNKNSFVGWSTDWSPYADQSIKVRISLKSALGDKAYEWNDNEMYLFRSSVAYAMRQYFLKVKNQMILFGEEDVRVANLKPRISFNFFVTAPKNVSDIIPRTEVEKAIRMSRSRINDAFRLNDNSLEFLGIQPTLGESKYGPPCPPCPAPEFLGGPSVFLFPPKPKDTLYITREPEVTCVVVDVSQEDPEVQFNWYVDGVEVHNAKTKPREEQFNSTYRVVSVLTVLHQDWLNGKEYKCKVSNKGLPSSIEKTISKAKGQPREPQVYTLPPSQEEMTKNQVSLTCLVKGFYPSDIAVEWESNGQPENNYKTTPPVLDSDGSFFLYSRLTVDKSRWQEGNVFSCSVMHEALHNHYTQKSLSLSLGK

SEQ ID NO: 36 - protein, 942 aa, synthetic construct
  REGION 1..723: note = ACE2 18-732 Q325P IgG1 YTE
QSTIEEQAKTFLDKFNHEAEDLFYQSSLASWNYNTNITEENVQNMNNAGDKWSAFLKEQSTLAQMYPLQEIQNLTVKLQLQALQQNGSSVLSEDKSKRLNTILNTMSTIYSTGKVCNPDNPQECLLLEPGLNEIMANSLDYNERLWAWESWRSEVGKQLRPLYEEYVVLKNEMARANHYEDYGDYWRGDYEVNGVDGYDYSRGQLIEDVEHTFEEIKPLYEHLHAYVRAKLMNAYPSYISPIGCLPAHLLGDMWGRFWTNLYSLTVPFGQKPNIDVTDAMVDQAWDAQRIFKEAEKFFVSVGLPNMTPGFWENSMLTDPGNVQKAVCHPTAWDLGKGDFRILMCTKVTMDDFLTAHHEMGHIQYDMAYAAQPFLLRNGANEGFHEAVGEIMSLSAATPKHLKSIGLLSPDFQEDNETEINFLLKQALTIVGTLPFTYMLEKWRWMVFKGEIPKDQWMKKWWEMKREIVGVVEPVPHDETYCDPASLFHVSNDYSFIRYYTRTLYQFQFQEALCQAAKHEGPLHKCDISNSTEAGQKLFNMLRLGKSEPWTLALENVVGAKNMNVRPLLNYFEPLFTWLKDQNKNSFVGWSTDWSPYADQSIKVRISLKSALGDKAYEWNDNEMYLFRSSVAYAMRQYFLKVKNQMILFGEEDVRVANLKPRISFNFFVTAPKNVSDIIPRTEVEKAIRMSRSRINDAFRLNDNSLEFLGIQPTLGDKTHTCPPCPAPELLGGPSVFLFPPKPKDTLYITREPEVTCVVVDVSHEDPEVKFNWYVDGVEVHNAKTKPREEQYNSTYRVVSVLTVLHQDWLNGKEYKCKVSNKALPAPIEKTISKAKGQPREPQVYTLPPSRDELTKNQVSLTCLVKGFYPSDIAVEWESNGQPENNYKTTPPVLDSDGSFFLYSKLTVDKSRWQQGNVFSCSVMHEALHNHYTQKSLSLSPGK

SEQ ID NO: 37 - protein, 944 aa, synthetic construct
  REGION 1..944: note = ACE2 18-732 Q325P IgG4 T256D T307Q
QSTIEEQAKTFLDKFNHEAEDLFYQSSLASWNYNTNITEENVQNMNNAGDKWSAFLKEQSTLAQMYPLQEIQNLTVKLQLQALQQNGSSVLSEDKSKRLNTILNTMSTIYSTGKVCNPDNPQECLLLEPGLNEIMANSLDYNERLWAWESWRSEVGKQLRPLYEEYVVLKNEMARANHYEDYGDYWRGDYEVNGVDGYDYSRGQLIEDVEHTFEEIKPLYEHLHAYVRAKLMNAYPSYISPIGCLPAHLLGDMWGRFWTNLYSLTVPFGQKPNIDVTDAMVDQAWDAQRIFKEAEKFFVSVGLPNMTPGFWENSMLTDPGNVQKAVCHPTAWDLGKGDFRILMCTKVTMDDFLTAHHEMGHIQYDMAYAAQPFLLRNGANEGFHEAVGEIMSLSAATPKHLKSIGLLSPDFQEDNETEINFLLKQALTIVGTLPFTYMLEKWRWMVFKGEIPKDQWMKKWWEMKREIVGVVEPVPHDETYCDPASLFHVSNDYSFIRYYTRTLYQFQFQEALCQAAKHEGPLHKCDISNSTEAGQKLFNMLRLGKSEPWTLALENVVGAKNMNVRPLLNYFEPLFTWLKDQNKNSFVGWSTDWSPYADQSIKVRISLKSALGDKAYEWNDNEMYLFRSSVAYAMRQYFLKVKNQMILFGEEDVRVANLKPRISFNFFVTAPKNVSDIIPRTEVEKAIRMSRSRINDAFRLNDNSLEFLGIQPTLGESKYGPPCPPCPAPEFLGGPSVFLFPPKPKDTLMISRDPEVTCVVVDVSQEDPEVQFNWYVDGVEVHNAKTKPREEQFNSTYRVVSVLQVLHQDWLNGKEYKCKVSNKGLPSSIEKTISKAKGQPREPQVYTLPPSQEEMTKNQVSLTCLVKGFYPSDIAVEWESNGQPENNYKTTPPVLDSDGSFFLYSRLTVDKSRWQEGNVFSCSVMHEALHNHYTQKSLSLSLGK

SEQ ID NO: 38 - protein, 942 aa, synthetic construct
  REGION 1..942: note = ACE2 18-732 Q325P IgG1 T256D T307Q
QSTIEEQAKTFLDKFNHEAEDLFYQSSLASWNYNTNITEENVQNMNNAGDKWSAFLKEQSTLAQMYPLQEIQNLTVKLQLQALQQNGSSVLSEDKSKRLNTILNTMSTIYSTGKVCNPDNPQECLLLEPGLNEIMANSLDYNERLWAWESWRSEVGKQLRPLYEEYVVLKNEMARANHYEDYGDYWRGDYEVNGVDGYDYSRGQLIEDVEHTFEEIKPLYEHLHAYVRAKLMNAYPSYISPIGCLPAHLLGDMWGRFWTNLYSLTVPFGQKPNIDVTDAMVDQAWDAQRIFKEAEKFFVSVGLPNMTPGFWENSMLTDPGNVQKAVCHPTAWDLGKGDFRILMCTKVTMDDFLTAHHEMGHIQYDMAYAAQPFLLRNGANEGFHEAVGEIMSLSAATPKHLKSIGLLSPDFQEDNETEINFLLKQALTIVGTLPFTYMLEKWRWMVFKGEIPKDQWMKKWWEMKREIVGVVEPVPHDETYCDPASLFHVSNDYSFIRYYTRTLYQFQFQEALCQAAKHEGPLHKCDISNSTEAGQKLFNMLRLGKSEPWTLALENVVGAKNMNVRPLLNYFEPLFTWLKDQNKNSFVGWSTDWSPYADQSIKVRISLKSALGDKAYEWNDNEMYLFRSSVAYAMRQYFLKVKNQMILFGEEDVRVANLKPRISFNFFVTAPKNVSDIIPRTEVEKAIRMSRSRINDAFRLNDNSLEFLGIQPTLGDKTHTCPPCPAPELLGGPSVFLFPPKPKDTLMISRDPEVTCVVVDVSHEDPEVKFNWYVDGVEVHNAKTKPREEQYNSTYRVVSVLQVLHQDWLNGKEYKCKVSNKALPAPIEKTISKAKGQPREPQVYTLPPSRDELTKNQVSLTCLVKGFYPSDIAVEWESNGQPENNYKTTPPVLDSDGSFFLYSKLTVDKSRWQQGNVFSCSVMHEALHNHYTQKSLSLSPGK

SEQ ID NO: 39 - protein, 944 aa, synthetic construct
  REGION 1..944: note = ACE2 18-732 T27A S645C IgG4 YTE
QSTIEEQAKAFLDKFNHEAEDLFYQSSLASWNYNTNITEENVQNMNNAGDKWSAFLKEQSTLAQMYPLQEIQNLTVKLQLQALQQNGSSVLSEDKSKRLNTILNTMSTIYSTGKVCNPDNPQECLLLEPGLNEIMANSLDYNERLWAWESWRSEVGKQLRPLYEEYVVLKNEMARANHYEDYGDYWRGDYEVNGVDGYDYSRGQLIEDVEHTFEEIKPLYEHLHAYVRAKLMNAYPSYISPIGCLPAHLLGDMWGRFWTNLYSLTVPFGQKPNIDVTDAMVDQAWDAQRIFKEAEKFFVSVGLPNMTQGFWENSMLTDPGNVQKAVCHPTAWDLGKGDFRILMCTKVTMDDFLTAHHEMGHIQYDMAYAAQPFLLRNGANEGFHEAVGEIMSLSAATPKHLKSIGLLSPDFQEDNETEINFLLKQALTIVGTLPFTYMLEKWRWMVFKGEIPKDQWMKKWWEMKREIVGVVEPVPHDETYCDPASLFHVSNDYSFIRYYTRTLYQFQFQEALCQAAKHEGPLHKCDISNSTEAGQKLFNMLRLGKSEPWTLALENVVGAKNMNVRPLLNYFEPLFTWLKDQNKNSFVGWSTDWSPYADQSIKVRISLKSALGDKAYEWNDNEMYLFRCSVAYAMRQYFLKVKNQMILFGEEDVRVANLKPRISFNFFVTAPKNVSDIIPRTEVEKAIRMSRSRINDAFRLNDNSLEFLGIQPTLGESKYGPPCPPCPAPEFLGGPSVFLFPPKPKDTLYITREPEVTCVVVDVSQEDPEVQFNWYVDGVEVHNAKTKPREEQFNSTYRVVSVLTVLHQDWLNGKEYKCKVSNKGLPSSIEKTISKAKGQPREPQVYTLPPSQEEMTKNQVSLTCLVKGFYPSDIAVEWESNGQPENNYKTTPPVLDSDGSFFLYSRLTVDKSRWQEGNVFSCSVMHEALHNHYTQKSLSLSLGK

SEQ ID NO: 40 - protein, 942 aa, synthetic construct
  REGION 1..942: note = ACE2 18-732 T27A S645C IgG1 YTE
QSTIEEQAKAFLDKFNHEAEDLFYQSSLASWNYNTNITEENVQNMNNAGDKWSAFLKEQSTLAQMYPLQEIQNLTVKLQLQALQQNGSSVLSEDKSKRLNTILNTMSTIYSTGKVCNPDNPQECLLLEPGLNEIMANSLDYNERLWAWESWRSEVGKQLRPLYEEYVVLKNEMARANHYEDYGDYWRGDYEVNGVDGYDYSRGQLIEDVEHTFEEIKPLYEHLHAYVRAKLMNAYPSYISPIGCLPAHLLGDMWGRFWTNLYSLTVPFGQKPNIDVTDAMVDQAWDAQRIFKEAEKFFVSVGLPNMTQGFWENSMLTDPGNVQKAVCHPTAWDLGKGDFRILMCTKVTMDDFLTAHHEMGHIQYDMAYAAQPFLLRNGANEGFHEAVGEIMSLSAATPKHLKSIGLLSPDFQEDNETEINFLLKQALTIVGTLPFTYMLEKWRWMVFKGEIPKDQWMKKWWEMKREIVGVVEPVPHDETYCDPASLFHVSNDYSFIRYYTRTLYQFQFQEALCQAAKHEGPLHKCDISNSTEAGQKLFNMLRLGKSEPWTLALENVVGAKNMNVRPLLNYFEPLFTWLKDQNKNSFVGWSTDWSPYADQSIKVRISLKSALGDKAYEWNDNEMYLFRCSVAYAMRQYFLKVKNQMILFGEEDVRVANLKPRISFNFFVTAPKNVSDIIPRTEVEKAIRMSRSRINDAFRLNDNSLEFLGIQPTLGDKTHTCPPCPAPELLGGPSVFLFPPKPKDTLYITREPEVTCVVVDVSHEDPEVKFNWYVDGVEVHNAKTKPREEQYNSTYRVVSVLTVLHQDWLNGKEYKCKVSNKALPAPIEKTISKAKGQPREPQVYTLPPSRDELTKNQVSLTCLVKGFYPSDIAVEWESNGQPENNYKTTPPVLDSDGSFFLYSKLTVDKSRWQQGNVFSCSVMHEALHNHYTQKSLSLSPGK

SEQ ID NO: 41 - protein, 944 aa, synthetic construct
  REGION 1..944: note = ACE2 18-732 T27A S645C IgG4 T256D T307Q
QSTIEEQAKAFLDKFNHEAEDLFYQSSLASWNYNTNITEENVQNMNNAGDKWSAFLKEQSTLAQMYPLQEIQNLTVKLQLQALQQNGSSVLSEDKSKRLNTILNTMSTIYSTGKVCNPDNPQECLLLEPGLNEIMANSLDYNERLWAWESWRSEVGKQLRPLYEEYVVLKNEMARANHYEDYGDYWRGDYEVNGVDGYDYSRGQLIEDVEHTFEEIKPLYEHLHAYVRAKLMNAYPSYISPIGCLPAHLLGDMWGRFWTNLYSLTVPFGQKPNIDVTDAMVDQAWDAQRIFKEAEKFFVSVGLPNMTQGFWENSMLTDPGNVQKAVCHPTAWDLGKGDFRILMCTKVTMDDFLTAHHEMGHIQYDMAYAAQPFLLRNGANEGFHEAVGEIMSLSAATPKHLKSIGLLSPDFQEDNETEINFLLKQALTIVGTLPFTYMLEKWRWMVFKGEIPKDQWMKKWWEMKREIVGVVEPVPHDETYCDPASLFHVSNDYSFIRYYTRTLYQFQFQEALCQAAKHEGPLHKCDISNSTEAGQKLFNMLRLGKSEPWTLALENVVGAKNMNVRPLLNYFEPLFTWLKDQNKNSFVGWSTDWSPYADQSIKVRISLKSALGDKAYEWNDNEMYLFRCSVAYAMRQYFLKVKNQMILFGEEDVRVANLKPRISFNFFVTAPKNVSDIIPRTEVEKAIRMSRSRINDAFRLNDNSLEFLGIQPTLGESKYGPPCPPCPAPEFLGGPSVFLFPPKPKDTLMISRDPEVTCVVVDVSQEDPEVQFNWYVDGVEVHNAKTKPREEQFNSTYRVVSVLQVLHQDWLNGKEYKCKVSNKGLPSSIEKTISKAKGQPREPQVYTLPPSQEEMTKNQVSLTCLVKGFYPSDIAVEWESNGQPENNYKTTPPVLDSDGSFFLYSRLTVDKSRWQEGNVFSCSVMHEALHNHYTQKSLSLSLGK

SEQ ID NO: 42 - protein, 942 aa, synthetic construct
  REGION 1..942: note = ACE2 18-732 T27A S645C IgG1 T256D T307Q
QSTIEEQAKAFLDKFNHEAEDLFYQSSLASWNYNTNITEENVQNMNNAGDKWSAFLKEQSTLAQMYPLQEIQNLTVKLQLQALQQNGSSVLSEDKSKRLNTILNTMSTIYSTGKVCNPDNPQECLLLEPGLNEIMANSLDYNERLWAWESWRSEVGKQLRPLYEEYVVLKNEMARANHYEDYGDYWRGDYEVNGVDGYDYSRGQLIEDVEHTFEEIKPLYEHLHAYVRAKLMNAYPSYISPIGCLPAHLLGDMWGRFWTNLYSLTVPFGQKPNIDVTDAMVDQAWDAQRIFKEAEKFFVSVGLPNMTQGFWENSMLTDPGNVQKAVCHPTAWDLGKGDFRILMCTKVTMDDFLTAHHEMGHIQYDMAYAAQPFLLRNGANEGFHEAVGEIMSLSAATPKHLKSIGLLSPDFQEDNETEINFLLKQALTIVGTLPFTYMLEKWRWMVFKGEIPKDQWMKKWWEMKREIVGVVEPVPHDETYCDPASLFHVSNDYSFIRYYTRTLYQFQFQEALCQAAKHEGPLHKCDISNSTEAGQKLFNMLRLGKSEPWTLALENVVGAKNMNVRPLLNYFEPLFTWLKDQNKNSFVGWSTDWSPYADQSIKVRISLKSALGDKAYEWNDNEMYLFRCSVAYAMRQYFLKVKNQMILFGEEDVRVANLKPRISFNFFVTAPKNVSDIIPRTEVEKAIRMSRSRINDAFRLNDNSLEFLGIQPTLGDKTHTCPPCPAPELLGGPSVFLFPPKPKDTLMISRDPEVTCVVVDVSHEDPEVKFNWYVDGVEVHNAKTKPREEQYNSTYRVVSVLQVLHQDWLNGKEYKCKVSNKALPAPIEKTISKAKGQPREPQVYTLPPSRDELTKNQVSLTCLVKGFYPSDIAVEWESNGQPENNYKTTPPVLDSDGSFFLYSKLTVDKSRWQQGNVFSCSVMHEALHNHYTQKSLSLSPGK

SEQ ID NO: 43 - protein, 944 aa, synthetic construct
  REGION 1..944: note = ACE2 18-732 T92I S645C IgG4 YTE
QSTIEEQAKTFLDKFNHEAEDLFYQSSLASWNYNTNITEENVQNMNNAGDKWSAFLKEQSTLAQMYPLQEIQNLIVKLQLQALQQNGSSVLSEDKSKRLNTILNTMSTIYSTGKVCNPDNPQECLLLEPGLNEIMANSLDYNERLWAWESWRSEVGKQLRPLYEEYVVLKNEMARANHYEDYGDYWRGDYEVNGVDGYDYSRGQLIEDVEHTFEEIKPLYEHLHAYVRAKLMNAYPSYISPIGCLPAHLLGDMWGRFWTNLYSLTVPFGQKPNIDVTDAMVDQAWDAQRIFKEAEKFFVSVGLPNMTQGFWENSMLTDPGNVQKAVCHPTAWDLGKGDFRILMCTKVTMDDFLTAHHEMGHIQYDMAYAAQPFLLRNGANEGFHEAVGEIMSLSAATPKHLKSIGLLSPDFQEDNETEINFLLKQALTIVGTLPFTYMLEKWRWMVFKGEIPKDQWMKKWWEMKREIVGVVEPVPHDETYCDPASLFHVSNDYSFIRYYTRTLYQFQFQEALCQAAKHEGPLHKCDISNSTEAGQKLFNMLRLGKSEPWTLALENVVGAKNMNVRPLLNYFEPLFTWLKDQNKNSFVGWSTDWSPYADQSIKVRISLKSALGDKAYEWNDNEMYLFRCSVAYAMRQYFLKVKNQMILFGEEDVRVANLKPRISFNFFVTAPKNVSDIIPRTEVEKAIRMSRSRINDAFRLNDNSLEFLGIQPTLGESKYGPPCPPCPAPEFLGGPSVFLFPPKPKDTLYITREPEVTCVVVDVSQEDPEVQFNWYVDGVEVHNAKTKPREEQFNSTYRVVSVLTVLHQDWLNGKEYKCKVSNKGLPSSIEKTISKAKGQPREPQVYTLPPSQEEMTKNQVSLTCLVKGFYPSDIAVEWESNGQPENNYKTTPPVLDSDGSFFLYSRLTVDKSRWQEGNVFSCSVMHEALHNHYTQKSLSLSLGK

SEQ ID NO: 44 - protein, 942 aa, synthetic construct
  REGION 1..942: note = ACE2 18-732 T92I S645C IgG1 YTE
QSTIEEQAKTFLDKFNHEAEDLFYQSSLASWNYNTNITEENVQNMNNAGDKWSAFLKEQSTLAQMYPLQEIQNLIVKLQLQALQQNGSSVLSEDKSKRLNTILNTMSTIYSTGKVCNPDNPQECLLLEPGLNEIMANSLDYNERLWAWESWRSEVGKQLRPLYEEYVVLKNEMARANHYEDYGDYWRGDYEVNGVDGYDYSRGQLIEDVEHTFEEIKPLYEHLHAYVRAKLMNAYPSYISPIGCLPAHLLGDMWGRFWTNLYSLTVPFGQKPNIDVTDAMVDQAWDAQRIFKEAEKFFVSVGLPNMTQGFWENSMLTDPGNVQKAVCHPTAWDLGKGDFRILMCTKVTMDDFLTAHHEMGHIQYDMAYAAQPFLLRNGANEGFHEAVGEIMSLSAATPKHLKSIGLLSPDFQEDNETEINFLLKQALTIVGTLPFTYMLEKWRWMVFKGEIPKDQWMKKWWEMKREIVGVVEPVPHDETYCDPASLFHVSNDYSFIRYYTRTLYQFQFQEALCQAAKHEGPLHKCDISNSTEAGQKLFNMLRLGKSEPWTLALENVVGAKNMNVRPLLNYFEPLFTWLKDQNKNSFVGWSTDWSPYADQSIKVRISLKSALGDKAYEWNDNEMYLFRCSVAYAMRQYFLKVKNQMILFGEEDVRVANLKPRISFNFFVTAPKNVSDIIPRTEVEKAIRMSRSRINDAFRLNDNSLEFLGIQPTLGDKTHTCPPCPAPELLGGPSVFLFPPKPKDTLYITREPEVTCVVVDVSHEDPEVKFNWYVDGVEVHNAKTKPREEQYNSTYRVVSVLTVLHQDWLNGKEYKCKVSNKALPAPIEKTISKAKGQPREPQVYTLPPSRDELTKNQVSLTCLVKGFYPSDIAVEWESNGQPENNYKTTPPVLDSDGSFFLYSKLTVDKSRWQQGNVFSCSVMHEALHNHYTQKSLSLSPGK

SEQ ID NO: 45 - protein, 944 aa, synthetic construct
  REGION 1..944: note = ACE2 18-732 T92I S645C IgG4 T256D T307Q
QSTIEEQAKTFLDKFNHEAEDLFYQSSLASWNYNTNITEENVQNMNNAGDKWSAFLKEQSTLAQMYPLQEIQNLIVKLQLQALQQNGSSVLSEDKSKRLNTILNTMSTIYSTGKVCNPDNPQECLLLEPGLNEIMANSLDYNERLWAWESWRSEVGKQLRPLYEEYVVLKNEMARANHYEDYGDYWRGDYEVNGVDGYDYSRGQLIEDVEHTFEEIKPLYEHLHAYVRAKLMNAYPSYISPIGCLPAHLLGDMWGRFWTNLYSLTVPFGQKPNIDVTDAMVDQAWDAQRIFKEAEKFFVSVGLPNMTQGFWENSMLTDPGNVQKAVCHPTAWDLGKGDFRILMCTKVTMDDFLTAHHEMGHIQYDMAYAAQPFLLRNGANEGFHEAVGEIMSLSAATPKHLKSIGLLSPDFQEDNETEINFLLKQALTIVGTLPFTYMLEKWRWMVFKGEIPKDQWMKKWWEMKREIVGVVEPVPHDETYCDPASLFHVSNDYSFIRYYTRTLYQFQFQEALCQAAKHEGPLHKCDISNSTEAGQKLFNMLRLGKSEPWTLALENVVGAKNMNVRPLLNYFEPLFTWLKDQNKNSFVGWSTDWSPYADQSIKVRISLKSALGDKAYEWNDNEMYLFRCSVAYAMRQYFLKVKNQMILFGEEDVRVANLKPRISFNFFVTAPKNVSDIIPRTEVEKAIRMSRSRINDAFRLNDNSLEFLGIQPTLGESKYGPPCPPCPAPEFLGGPSVFLFPPKPKDTLMISRDPEVTCVVVDVSQEDPEVQFNWYVDGVEVHNAKTKPREEQFNSTYRVVSVLQVLHQDWLNGKEYKCKVSNKGLPSSIEKTISKAKGQPREPQVYTLPPSQEEMTKNQVSLTCLVKGFYPSDIAVEWESNGQPENNYKTTPPVLDSDGSFFLYSRLTVDKSRWQEGNVFSCSVMHEALHNHYTQKSLSLSLGK

SEQ ID NO: 46 - protein, 942 aa, synthetic construct
  REGION 1..942: note = ACE2 18-732 T92I S645C IgG1 T256D T307Q
QSTIEEQAKTFLDKFNHEAEDLFYQSSLASWNYNTNITEENVQNMNNAGDKWSAFLKEQSTLAQMYPLQEIQNLIVKLQLQALQQNGSSVLSEDKSKRLNTILNTMSTIYSTGKVCNPDNPQECLLLEPGLNEIMANSLDYNERLWAWESWRSEVGKQLRPLYEEYVVLKNEMARANHYEDYGDYWRGDYEVNGVDGYDYSRGQLIEDVEHTFEEIKPLYEHLHAYVRAKLMNAYPSYISPIGCLPAHLLGDMWGRFWTNLYSLTVPFGQKPNIDVTDAMVDQAWDAQRIFKEAEKFFVSVGLPNMTQGFWENSMLTDPGNVQKAVCHPTAWDLGKGDFRILMCTKVTMDDFLTAHHEMGHIQYDMAYAAQPFLLRNGANEGFHEAVGEIMSLSAATPKHLKSIGLLSPDFQEDNETEINFLLKQALTIVGTLPFTYMLEKWRWMVFKGEIPKDQWMKKWWEMKREIVGVVEPVPHDETYCDPASLFHVSNDYSFIRYYTRTLYQFQFQEALCQAAKHEGPLHKCDISNSTEAGQKLFNMLRLGKSEPWTLALENVVGAKNMNVRPLLNYFEPLFTWLKDQNKNSFVGWSTDWSPYADQSIKVRISLKSALGDKAYEWNDNEMYLFRCSVAYAMRQYFLKVKNQMILFGEEDVRVANLKPRISFNFFVTAPKNVSDIIPRTEVEKAIRMSRSRINDAFRLNDNSLEFLGIQPTLGDKTHTCPPCPAPELLGGPSVFLFPPKPKDTLMISRDPEVTCVVVDVSHEDPEVKFNWYVDGVEVHNAKTKPREEQYNSTYRVVSVLQVLHQDWLNGKEYKCKVSNKALPAPIEKTISKAKGQPREPQVYTLPPSRDELTKNQVSLTCLVKGFYPSDIAVEWESNGQPENNYKTTPPVLDSDGSFFLYSKLTVDKSRWQQGNVFSCSVMHEALHNHYTQKSLSLSPGK

SEQ ID NO: 47 - protein, 944 aa, synthetic construct
  REGION 1..944: note = ACE2 18-732 Q325P S645C IgG4 YTE
QSTIEEQAKTFLDKFNHEAEDLFYQSSLASWNYNTNITEENVQNMNNAGDKWSAFLKEQSTLAQMYPLQEIQNLTVKLQLQALQQNGSSVLSEDKSKRLNTILNTMSTIYSTGKVCNPDNPQECLLLEPGLNEIMANSLDYNERLWAWESWRSEVGKQLRPLYEEYVVLKNEMARANHYEDYGDYWRGDYEVNGVDGYDYSRGQLIEDVEHTFEEIKPLYEHLHAYVRAKLMNAYPSYISPIGCLPAHLLGDMWGRFWTNLYSLTVPFGQKPNIDVTDAMVDQAWDAQRIFKEAEKFFVSVGLPNMTPGFWENSMLTDPGNVQKAVCHPTAWDLGKGDFRILMCTKVTMDDFLTAHHEMGHIQYDMAYAAQPFLLRNGANEGFHEAVGEIMSLSAATPKHLKSIGLLSPDFQEDNETEINFLLKQALTIVGTLPFTYMLEKWRWMVFKGEIPKDQWMKKWWEMKREIVGVVEPVPHDETYCDPASLFHVSNDYSFIRYYTRTLYQFQFQEALCQAAKHEGPLHKCDISNSTEAGQKLFNMLRLGKSEPWTLALENVVGAKNMNVRPLLNYFEPLFTWLKDQNKNSFVGWSTDWSPYADQSIKVRISLKSALGDKAYEWNDNEMYLFRCSVAYAMRQYFLKVKNQMILFGEEDVRVANLKPRISFNFFVTAPKNVSDIIPRTEVEKAIRMSRSRINDAFRLNDNSLEFLGIQPTLGESKYGPPCPPCPAPEFLGGPSVFLFPPKPKDTLYITREPEVTCVVVDVSQEDPEVQFNWYVDGVEVHNAKTKPREEQFNSTYRVVSVLTVLHQDWLNGKEYKCKVSNKGLPSSIEKTISKAKGQPREPQVYTLPPSQEEMTKNQVSLTCLVKGFYPSDIAVEWESNGQPENNYKTTPPVLDSDGSFFLYSRLTVDKSRWQEGNVFSCSVMHEALHNHYTQKSLSLSLGK

SEQ ID NO: 48 - protein, 942 aa, synthetic construct
  REGION 1..942: note = ACE2 18-732 Q325P S645C IgG1 YTE
QSTIEEQAKTFLDKFNHEAEDLFYQSSLASWNYNTNITEENVQNMNNAGDKWSAFLKEQSTLAQMYPLQEIQNLTVKLQLQALQQNGSSVLSEDKSKRLNTILNTMSTIYSTGKVCNPDNPQECLLLEPGLNEIMANSLDYNERLWAWESWRSEVGKQLRPLYEEYVVLKNEMARANHYEDYGDYWRGDYEVNGVDGYDYSRGQLIEDVEHTFEEIKPLYEHLHAYVRAKLMNAYPSYISPIGCLPAHLLGDMWGRFWTNLYSLTVPFGQKPNIDVTDAMVDQAWDAQRIFKEAEKFFVSVGLPNMTPGFWENSMLTDPGNVQKAVCHPTAWDLGKGDFRILMCTKVTMDDFLTAHHEMGHIQYDMAYAAQPFLLRNGANEGFHEAVGEIMSLSAATPKHLKSIGLLSPDFQEDNETEINFLLKQALTIVGTLPFTYMLEKWRWMVFKGEIPKDQWMKKWWEMKREIVGVVEPVPHDETYCDPASLFHVSNDYSFIRYYTRTLYQFQFQEALCQAAKHEGPLHKCDISNSTEAGQKLFNMLRLGKSEPWTLALENVVGAKNMNVRPLLNYFEPLFTWLKDQNKNSFVGWSTDWSPYADQSIKVRISLKSALGDKAYEWNDNEMYLFRCSVAYAMRQYFLKVKNQMILFGEEDVRVANLKPRISFNFFVTAPKNVSDIIPRTEVEKAIRMSRSRINDAFRLNDNSLEFLGIQPTLGDKTHTCPPCPAPELLGGPSVFLFPPKPKDTLYITREPEVTCVVVDVSHEDPEVKFNWYVDGVEVHNAKTKPREEQYNSTYRVVSVLTVLHQDWLNGKEYKCKVSNKALPAPIEKTISKAKGQPREPQVYTLPPSRDELTKNQVSLTCLVKGFYPSDIAVEWESNGQPENNYKTTPPVLDSDGSFFLYSKLTVDKSRWQQGNVFSCSVMHEALHNHYTQKSLSLSPGK

SEQ ID NO: 49 - protein, 944 aa, synthetic construct
  REGION 1..715: note = ACE2 18-732 Q325P S645C IgG4 T256D T307Q
QSTIEEQAKTFLDKFNHEAEDLFYQSSLASWNYNTNITEENVQNMNNAGDKWSAFLKEQSTLAQMYPLQEIQNLTVKLQLQALQQNGSSVLSEDKSKRLNTILNTMSTIYSTGKVCNPDNPQECLLLEPGLNEIMANSLDYNERLWAWESWRSEVGKQLRPLYEEYVVLKNEMARANHYEDYGDYWRGDYEVNGVDGYDYSRGQLIEDVEHTFEEIKPLYEHLHAYVRAKLMNAYPSYISPIGCLPAHLLGDMWGRFWTNLYSLTVPFGQKPNIDVTDAMVDQAWDAQRIFKEAEKFFVSVGLPNMTPGFWENSMLTDPGNVQKAVCHPTAWDLGKGDFRILMCTKVTMDDFLTAHHEMGHIQYDMAYAAQPFLLRNGANEGFHEAVGEIMSLSAATPKHLKSIGLLSPDFQEDNETEINFLLKQALTIVGTLPFTYMLEKWRWMVFKGEIPKDQWMKKWWEMKREIVGVVEPVPHDETYCDPASLFHVSNDYSFIRYYTRTLYQFQFQEALCQAAKHEGPLHKCDISNSTEAGQKLFNMLRLGKSEPWTLALENVVGAKNMNVRPLLNYFEPLFTWLKDQNKNSFVGWSTDWSPYADQSIKVRISLKSALGDKAYEWNDNEMYLFRCSVAYAMRQYFLKVKNQMILFGEEDVRVANLKPRISFNFFVTAPKNVSDIIPRTEVEKAIRMSRSRINDAFRLNDNSLEFLGIQPTLGESKYGPPCPPCPAPEFLGGPSVFLFPPKPKDTLMISRDPEVTCVVVDVSQEDPEVQFNWYVDGVEVHNAKTKPREEQFNSTYRVVSVLQVLHQDWLNGKEYKCKVSNKGLPSSIEKTISKAKGQPREPQVYTLPPSQEEMTKNQVSLTCLVKGFYPSDIAVEWESNGQPENNYKTTPPVLDSDGSFFLYSRLTVDKSRWQEGNVFSCSVMHEALHNHYTQKSLSLSLGK

SEQ ID NO: 50 - protein, 942 aa, synthetic construct
  REGION 1..723: note = ACE2 18-732 Q325P S645C IgG1 T256D T307Q
QSTIEEQAKTFLDKFNHEAEDLFYQSSLASWNYNTNITEENVQNMNNAGDKWSAFLKEQSTLAQMYPLQEIQNLTVKLQLQALQQNGSSVLSEDKSKRLNTILNTMSTIYSTGKVCNPDNPQECLLLEPGLNEIMANSLDYNERLWAWESWRSEVGKQLRPLYEEYVVLKNEMARANHYEDYGDYWRGDYEVNGVDGYDYSRGQLIEDVEHTFEEIKPLYEHLHAYVRAKLMNAYPSYISPIGCLPAHLLGDMWGRFWTNLYSLTVPFGQKPNIDVTDAMVDQAWDAQRIFKEAEKFFVSVGLPNMTPGFWENSMLTDPGNVQKAVCHPTAWDLGKGDFRILMCTKVTMDDFLTAHHEMGHIQYDMAYAAQPFLLRNGANEGFHEAVGEIMSLSAATPKHLKSIGLLSPDFQEDNETEINFLLKQALTIVGTLPFTYMLEKWRWMVFKGEIPKDQWMKKWWEMKREIVGVVEPVPHDETYCDPASLFHVSNDYSFIRYYTRTLYQFQFQEALCQAAKHEGPLHKCDISNSTEAGQKLFNMLRLGKSEPWTLALENVVGAKNMNVRPLLNYFEPLFTWLKDQNKNSFVGWSTDWSPYADQSIKVRISLKSALGDKAYEWNDNEMYLFRCSVAYAMRQYFLKVKNQMILFGEEDVRVANLKPRISFNFFVTAPKNVSDIIPRTEVEKAIRMSRSRINDAFRLNDNSLEFLGIQPTLGDKTHTCPPCPAPELLGGPSVFLFPPKPKDTLMISRDPEVTCVVVDVSHEDPEVKFNWYVDGVEVHNAKTKPREEQYNSTYRVVSVLQVLHQDWLNGKEYKCKVSNKALPAPIEKTISKAKGQPREPQVYTLPPSRDELTKNQVSLTCLVKGFYPSDIAVEWESNGQPENNYKTTPPVLDSDGSFFLYSKLTVDKSRWQQGNVFSCSVMHEALHNHYTQKSLSLSPGK

SEQ ID NO: 51 - protein, 944 aa, synthetic construct
  REGION 1..944: note = ACE2 18-732 T27A T92I S645C IgG4 YTE
QSTIEEQAKAFLDKFNHEAEDLFYQSSLASWNYNTNITEENVQNMNNAGDKWSAFLKEQSTLAQMYPLQEIQNLIVKLQLQALQQNGSSVLSEDKSKRLNTILNTMSTIYSTGKVCNPDNPQECLLLEPGLNEIMANSLDYNERLWAWESWRSEVGKQLRPLYEEYVVLKNEMARANHYEDYGDYWRGDYEVNGVDGYDYSRGQLIEDVEHTFEEIKPLYEHLHAYVRAKLMNAYPSYISPIGCLPAHLLGDMWGRFWTNLYSLTVPFGQKPNIDVTDAMVDQAWDAQRIFKEAEKFFVSVGLPNMTQGFWENSMLTDPGNVQKAVCHPTAWDLGKGDFRILMCTKVTMDDFLTAHHEMGHIQYDMAYAAQPFLLRNGANEGFHEAVGEIMSLSAATPKHLKSIGLLSPDFQEDNETEINFLLKQALTIVGTLPFTYMLEKWRWMVFKGEIPKDQWMKKWWEMKREIVGVVEPVPHDETYCDPASLFHVSNDYSFIRYYTRTLYQFQFQEALCQAAKHEGPLHKCDISNSTEAGQKLFNMLRLGKSEPWTLALENVVGAKNMNVRPLLNYFEPLFTWLKDQNKNSFVGWSTDWSPYADQSIKVRISLKSALGDKAYEWNDNEMYLFRCSVAYAMRQYFLKVKNQMILFGEEDVRVANLKPRISFNFFVTAPKNVSDIIPRTEVEKAIRMSRSRINDAFRLNDNSLEFLGIQPTLGESKYGPPCPPCPAPEFLGGPSVFLFPPKPKDTLYITREPEVTCVVVDVSQEDPEVQFNWYVDGVEVHNAKTKPREEQFNSTYRVVSVLTVLHQDWLNGKEYKCKVSNKGLPSSIEKTISKAKGQPREPQVYTLPPSQEEMTKNQVSLTCLVKGFYPSDIAVEWESNGQPENNYKTTPPVLDSDGSFFLYSRLTVDKSRWQEGNVFSCSVMHEALHNHYTQKSLSLSLGK

SEQ ID NO: 52 - protein, 942 aa, synthetic construct
  REGION 1..942: note = ACE2 18-732 T27A T92I S645C IgG1 YTE
QSTIEEQAKAFLDKFNHEAEDLFYQSSLASWNYNTNITEENVQNMNNAGDKWSAFLKEQSTLAQMYPLQEIQNLIVKLQLQALQQNGSSVLSEDKSKRLNTILNTMSTIYSTGKVCNPDNPQECLLLEPGLNEIMANSLDYNERLWAWESWRSEVGKQLRPLYEEYVVLKNEMARANHYEDYGDYWRGDYEVNGVDGYDYSRGQLIEDVEHTFEEIKPLYEHLHAYVRAKLMNAYPSYISPIGCLPAHLLGDMWGRFWTNLYSLTVPFGQKPNIDVTDAMVDQAWDAQRIFKEAEKFFVSVGLPNMTQGFWENSMLTDPGNVQKAVCHPTAWDLGKGDFRILMCTKVTMDDFLTAHHEMGHIQYDMAYAAQPFLLRNGANEGFHEAVGEIMSLSAATPKHLKSIGLLSPDFQEDNETEINFLLKQALTIVGTLPFTYMLEKWRWMVFKGEIPKDQWMKKWWEMKREIVGVVEPVPHDETYCDPASLFHVSNDYSFIRYYTRTLYQFQFQEALCQAAKHEGPLHKCDISNSTEAGQKLFNMLRLGKSEPWTLALENVVGAKNMNVRPLLNYFEPLFTWLKDQNKNSFVGWSTDWSPYADQSIKVRISLKSALGDKAYEWNDNEMYLFRCSVAYAMRQYFLKVKNQMILFGEEDVRVANLKPRISFNFFVTAPKNVSDIIPRTEVEKAIRMSRSRINDAFRLNDNSLEFLGIQPTLGDKTHTCPPCPAPELLGGPSVFLFPPKPKDTLYITREPEVTCVVVDVSHEDPEVKFNWYVDGVEVHNAKTKPREEQYNSTYRVVSVLTVLHQDWLNGKEYKCKVSNKALPAPIEKTISKAKGQPREPQVYTLPPSRDELTKNQVSLTCLVKGFYPSDIAVEWESNGQPENNYKTTPPVLDSDGSFFLYSKLTVDKSRWQQGNVFSCSVMHEALHNHYTQKSLSLSPGK

SEQ ID NO: 53 - protein, 944 aa, synthetic construct
  REGION 1..944: note = ACE2 18-732 T27A T92I S645C IgG4 T256D T307Q
QSTIEEQAKAFLDKFNHEAEDLFYQSSLASWNYNTNITEENVQNMNNAGDKWSAFLKEQSTLAQMYPLQEIQNLIVKLQLQALQQNGSSVLSEDKSKRLNTILNTMSTIYSTGKVCNPDNPQECLLLEPGLNEIMANSLDYNERLWAWESWRSEVGKQLRPLYEEYVVLKNEMARANHYEDYGDYWRGDYEVNGVDGYDYSRGQLIEDVEHTFEEIKPLYEHLHAYVRAKLMNAYPSYISPIGCLPAHLLGDMWGRFWTNLYSLTVPFGQKPNIDVTDAMVDQAWDAQRIFKEAEKFFVSVGLPNMTQGFWENSMLTDPGNVQKAVCHPTAWDLGKGDFRILMCTKVTMDDFLTAHHEMGHIQYDMAYAAQPFLLRNGANEGFHEAVGEIMSLSAATPKHLKSIGLLSPDFQEDNETEINFLLKQALTIVGTLPFTYMLEKWRWMVFKGEIPKDQWMKKWWEMKREIVGVVEPVPHDETYCDPASLFHVSNDYSFIRYYTRTLYQFQFQEALCQAAKHEGPLHKCDISNSTEAGQKLFNMLRLGKSEPWTLALENVVGAKNMNVRPLLNYFEPLFTWLKDQNKNSFVGWSTDWSPYADQSIKVRISLKSALGDKAYEWNDNEMYLFRCSVAYAMRQYFLKVKNQMILFGEEDVRVANLKPRISFNFFVTAPKNVSDIIPRTEVEKAIRMSRSRINDAFRLNDNSLEFLGIQPTLGESKYGPPCPPCPAPEFLGGPSVFLFPPKPKDTLMISRDPEVTCVVVDVSQEDPEVQFNWYVDGVEVHNAKTKPREEQFNSTYRVVSVLQVLHQDWLNGKEYKCKVSNKGLPSSIEKTISKAKGQPREPQVYTLPPSQEEMTKNQVSLTCLVKGFYPSDIAVEWESNGQPENNYKTTPPVLDSDGSFFLYSRLTVDKSRWQEGNVFSCSVMHEALHNHYTQKSLSLSLGK

SEQ ID NO: 54 - protein, 942 aa, synthetic construct
  REGION 1..942: note = ACE2 18-732 T27A T92I S645C IgG1 T256D T307Q
QSTIEEQAKAFLDKFNHEAEDLFYQSSLASWNYNTNITEENVQNMNNAGDKWSAFLKEQSTLAQMYPLQEIQNLIVKLQLQALQQNGSSVLSEDKSKRLNTILNTMSTIYSTGKVCNPDNPQECLLLEPGLNEIMANSLDYNERLWAWESWRSEVGKQLRPLYEEYVVLKNEMARANHYEDYGDYWRGDYEVNGVDGYDYSRGQLIEDVEHTFEEIKPLYEHLHAYVRAKLMNAYPSYISPIGCLPAHLLGDMWGRFWTNLYSLTVPFGQKPNIDVTDAMVDQAWDAQRIFKEAEKFFVSVGLPNMTQGFWENSMLTDPGNVQKAVCHPTAWDLGKGDFRILMCTKVTMDDFLTAHHEMGHIQYDMAYAAQPFLLRNGANEGFHEAVGEIMSLSAATPKHLKSIGLLSPDFQEDNETEINFLLKQALTIVGTLPFTYMLEKWRWMVFKGEIPKDQWMKKWWEMKREIVGVVEPVPHDETYCDPASLFHVSNDYSFIRYYTRTLYQFQFQEALCQAAKHEGPLHKCDISNSTEAGQKLFNMLRLGKSEPWTLALENVVGAKNMNVRPLLNYFEPLFTWLKDQNKNSFVGWSTDWSPYADQSIKVRISLKSALGDKAYEWNDNEMYLFRCSVAYAMRQYFLKVKNQMILFGEEDVRVANLKPRISFNFFVTAPKNVSDIIPRTEVEKAIRMSRSRINDAFRLNDNSLEFLGIQPTLGDKTHTCPPCPAPELLGGPSVFLFPPKPKDTLMISRDPEVTCVVVDVSHEDPEVKFNWYVDGVEVHNAKTKPREEQYNSTYRVVSVLQVLHQDWLNGKEYKCKVSNKALPAPIEKTISKAKGQPREPQVYTLPPSRDELTKNQVSLTCLVKGFYPSDIAVEWESNGQPENNYKTTPPVLDSDGSFFLYSKLTVDKSRWQQGNVFSCSVMHEALHNHYTQKSLSLSPGK

SEQ ID NO: 55 - protein, 944 aa, synthetic construct
  REGION 1..944: note = ACE2 18-732 T27A Q325P S645C IgG4 YTE
QSTIEEQAKAFLDKFNHEAEDLFYQSSLASWNYNTNITEENVQNMNNAGDKWSAFLKEQSTLAQMYPLQEIQNLTVKLQLQALQQNGSSVLSEDKSKRLNTILNTMSTIYSTGKVCNPDNPQECLLLEPGLNEIMANSLDYNERLWAWESWRSEVGKQLRPLYEEYVVLKNEMARANHYEDYGDYWRGDYEVNGVDGYDYSRGQLIEDVEHTFEEIKPLYEHLHAYVRAKLMNAYPSYISPIGCLPAHLLGDMWGRFWTNLYSLTVPFGQKPNIDVTDAMVDQAWDAQRIFKEAEKFFVSVGLPNMTPGFWENSMLTDPGNVQKAVCHPTAWDLGKGDFRILMCTKVTMDDFLTAHHEMGHIQYDMAYAAQPFLLRNGANEGFHEAVGEIMSLSAATPKHLKSIGLLSPDFQEDNETEINFLLKQALTIVGTLPFTYMLEKWRWMVFKGEIPKDQWMKKWWEMKREIVGVVEPVPHDETYCDPASLFHVSNDYSFIRYYTRTLYQFQFQEALCQAAKHEGPLHKCDISNSTEAGQKLFNMLRLGKSEPWTLALENVVGAKNMNVRPLLNYFEPLFTWLKDQNKNSFVGWSTDWSPYADQSIKVRISLKSALGDKAYEWNDNEMYLFRCSVAYAMRQYFLKVKNQMILFGEEDVRVANLKPRISFNFFVTAPKNVSDIIPRTEVEKAIRMSRSRINDAFRLNDNSLEFLGIQPTLGESKYGPPCPPCPAPEFLGGPSVFLFPPKPKDTLYITREPEVTCVVVDVSQEDPEVQFNWYVDGVEVHNAKTKPREEQFNSTYRVVSVLTVLHQDWLNGKEYKCKVSNKGLPSSIEKTISKAKGQPREPQVYTLPPSQEEMTKNQVSLTCLVKGFYPSDIAVEWESNGQPENNYKTTPPVLDSDGSFFLYSRLTVDKSRWQEGNVFSCSVMHEALHNHYTQKSLSLSLGK

SEQ ID NO: 56 - protein, 942 aa, synthetic construct
  REGION 1..942: note = ACE2 18-732 T27A Q325P S645C IgG1 YTE
QSTIEEQAKAFLDKFNHEAEDLFYQSSLASWNYNTNITEENVQNMNNAGDKWSAFLKEQSTLAQMYPLQEIQNLTVKLQLQALQQNGSSVLSEDKSKRLNTILNTMSTIYSTGKVCNPDNPQECLLLEPGLNEIMANSLDYNERLWAWESWRSEVGKQLRPLYEEYVVLKNEMARANHYEDYGDYWRGDYEVNGVDGYDYSRGQLIEDVEHTFEEIKPLYEHLHAYVRAKLMNAYPSYISPIGCLPAHLLGDMWGRFWTNLYSLTVPFGQKPNIDVTDAMVDQAWDAQRIFKEAEKFFVSVGLPNMTPGFWENSMLTDPGNVQKAVCHPTAWDLGKGDFRILMCTKVTMDDFLTAHHEMGHIQYDMAYAAQPFLLRNGANEGFHEAVGEIMSLSAATPKHLKSIGLLSPDFQEDNETEINFLLKQALTIVGTLPFTYMLEKWRWMVFKGEIPKDQWMKKWWEMKREIVGVVEPVPHDETYCDPASLFHVSNDYSFIRYYTRTLYQFQFQEALCQAAKHEGPLHKCDISNSTEAGQKLFNMLRLGKSEPWTLALENVVGAKNMNVRPLLNYFEPLFTWLKDQNKNSFVGWSTDWSPYADQSIKVRISLKSALGDKAYEWNDNEMYLFRCSVAYAMRQYFLKVKNQMILFGEEDVRVANLKPRISFNFFVTAPKNVSDIIPRTEVEKAIRMSRSRINDAFRLNDNSLEFLGIQPTLGDKTHTCPPCPAPELLGGPSVFLFPPKPKDTLYITREPEVTCVVVDVSHEDPEVKFNWYVDGVEVHNAKTKPREEQYNSTYRVVSVLTVLHQDWLNGKEYKCKVSNKALPAPIEKTISKAKGQPREPQVYTLPPSRDELTKNQVSLTCLVKGFYPSDIAVEWESNGQPENNYKTTPPVLDSDGSFFLYSKLTVDKSRWQQGNVFSCSVMHEALHNHYTQKSLSLSPGK

SEQ ID NO: 57 - protein, 944 aa, synthetic construct
  REGION 1..944: note = ACE2 18-732 T27A Q325P S645C IgG4 T256D T307Q
QSTIEEQAKAFLDKFNHEAEDLFYQSSLASWNYNTNITEENVQNMNNAGDKWSAFLKEQSTLAQMYPLQEIQNLTVKLQLQALQQNGSSVLSEDKSKRLNTILNTMSTIYSTGKVCNPDNPQECLLLEPGLNEIMANSLDYNERLWAWESWRSEVGKQLRPLYEEYVVLKNEMARANHYEDYGDYWRGDYEVNGVDGYDYSRGQLIEDVEHTFEEIKPLYEHLHAYVRAKLMNAYPSYISPIGCLPAHLLGDMWGRFWTNLYSLTVPFGQKPNIDVTDAMVDQAWDAQRIFKEAEKFFVSVGLPNMTPGFWENSMLTDPGNVQKAVCHPTAWDLGKGDFRILMCTKVTMDDFLTAHHEMGHIQYDMAYAAQPFLLRNGANEGFHEAVGEIMSLSAATPKHLKSIGLLSPDFQEDNETEINFLLKQALTIVGTLPFTYMLEKWRWMVFKGEIPKDQWMKKWWEMKREIVGVVEPVPHDETYCDPASLFHVSNDYSFIRYYTRTLYQFQFQEALCQAAKHEGPLHKCDISNSTEAGQKLFNMLRLGKSEPWTLALENVVGAKNMNVRPLLNYFEPLFTWLKDQNKNSFVGWSTDWSPYADQSIKVRISLKSALGDKAYEWNDNEMYLFRCSVAYAMRQYFLKVKNQMILFGEEDVRVANLKPRISFNFFVTAPKNVSDIIPRTEVEKAIRMSRSRINDAFRLNDNSLEFLGIQPTLGESKYGPPCPPCPAPEFLGGPSVFLFPPKPKDTLMISRDPEVTCVVVDVSQEDPEVQFNWYVDGVEVHNAKTKPREEQFNSTYRVVSVLQVLHQDWLNGKEYKCKVSNKGLPSSIEKTISKAKGQPREPQVYTLPPSQEEMTKNQVSLTCLVKGFYPSDIAVEWESNGQPENNYKTTPPVLDSDGSFFLYSRLTVDKSRWQEGNVFSCSVMHEALHNHYTQKSLSLSLGK

SEQ ID NO: 58 - protein, 942 aa, synthetic construct
  REGION 1..942: note = ACE2 18-732 T27A Q325P S645C IgG1 T256D T 307Q
QSTIEEQAKAFLDKFNHEAEDLFYQSSLASWNYNTNITEENVQNMNNAGDKWSAFLKEQSTLAQMYPLQEIQNLTVKLQLQALQQNGSSVLSEDKSKRLNTILNTMSTIYSTGKVCNPDNPQECLLLEPGLNEIMANSLDYNERLWAWESWRSEVGKQLRPLYEEYVVLKNEMARANHYEDYGDYWRGDYEVNGVDGYDYSRGQLIEDVEHTFEEIKPLYEHLHAYVRAKLMNAYPSYISPIGCLPAHLLGDMWGRFWTNLYSLTVPFGQKPNIDVTDAMVDQAWDAQRIFKEAEKFFVSVGLPNMTPGFWENSMLTDPGNVQKAVCHPTAWDLGKGDFRILMCTKVTMDDFLTAHHEMGHIQYDMAYAAQPFLLRNGANEGFHEAVGEIMSLSAATPKHLKSIGLLSPDFQEDNETEINFLLKQALTIVGTLPFTYMLEKWRWMVFKGEIPKDQWMKKWWEMKREIVGVVEPVPHDETYCDPASLFHVSNDYSFIRYYTRTLYQFQFQEALCQAAKHEGPLHKCDISNSTEAGQKLFNMLRLGKSEPWTLALENVVGAKNMNVRPLLNYFEPLFTWLKDQNKNSFVGWSTDWSPYADQSIKVRISLKSALGDKAYEWNDNEMYLFRCSVAYAMRQYFLKVKNQMILFGEEDVRVANLKPRISFNFFVTAPKNVSDIIPRTEVEKAIRMSRSRINDAFRLNDNSLEFLGIQPTLGDKTHTCPPCPAPELLGGPSVFLFPPKPKDTLMISRDPEVTCVVVDVSHEDPEVKFNWYVDGVEVHNAKTKPREEQYNSTYRVVSVLQVLHQDWLNGKEYKCKVSNKALPAPIEKTISKAKGQPREPQVYTLPPSRDELTKNQVSLTCLVKGFYPSDIAVEWESNGQPENNYKTTPPVLDSDGSFFLYSKLTVDKSRWQQGNVFSCSVMHEALHNHYTQKSLSLSPGK

SEQ ID NO: 59 - protein, 944 aa, synthetic construct
  REGION 1..944: note = ACE2 18-732 T92I Q325P S645C IgG4 YTE
QSTIEEQAKTFLDKFNHEAEDLFYQSSLASWNYNTNITEENVQNMNNAGDKWSAFLKEQSTLAQMYPLQEIQNLIVKLQLQALQQNGSSVLSEDKSKRLNTILNTMSTIYSTGKVCNPDNPQECLLLEPGLNEIMANSLDYNERLWAWESWRSEVGKQLRPLYEEYVVLKNEMARANHYEDYGDYWRGDYEVNGVDGYDYSRGQLIEDVEHTFEEIKPLYEHLHAYVRAKLMNAYPSYISPIGCLPAHLLGDMWGRFWTNLYSLTVPFGQKPNIDVTDAMVDQAWDAQRIFKEAEKFFVSVGLPNMTPGFWENSMLTDPGNVQKAVCHPTAWDLGKGDFRILMCTKVTMDDFLTAHHEMGHIQYDMAYAAQPFLLRNGANEGFHEAVGEIMSLSAATPKHLKSIGLLSPDFQEDNETEINFLLKQALTIVGTLPFTYMLEKWRWMVFKGEIPKDQWMKKWWEMKREIVGVVEPVPHDETYCDPASLFHVSNDYSFIRYYTRTLYQFQFQEALCQAAKHEGPLHKCDISNSTEAGQKLFNMLRLGKSEPWTLALENVVGAKNMNVRPLLNYFEPLFTWLKDQNKNSFVGWSTDWSPYADQSIKVRISLKSALGDKAYEWNDNEMYLFRCSVAYAMRQYFLKVKNQMILFGEEDVRVANLKPRISFNFFVTAPKNVSDIIPRTEVEKAIRMSRSRINDAFRLNDNSLEFLGIQPTLGESKYGPPCPPCPAPEFLGGPSVFLFPPKPKDTLYITREPEVTCVVVDVSQEDPEVQFNWYVDGVEVHNAKTKPREEQFNSTYRVVSVLTVLHQDWLNGKEYKCKVSNKGLPSSIEKTISKAKGQPREPQVYTLPPSQEEMTKNQVSLTCLVKGFYPSDIAVEWESNGQPENNYKTTPPVLDSDGSFFLYSRLTVDKSRWQEGNVFSCSVMHEALHNHYTQKSLSLSLGK

SEQ ID NO: 60 - protein, 942 aa, synthetic construct
  REGION 1..942: note = ACE2 18-732 T92I Q325P S645C IgG1 YTE
QSTIEEQAKTFLDKFNHEAEDLFYQSSLASWNYNTNITEENVQNMNNAGDKWSAFLKEQSTLAQMYPLQEIQNLIVKLQLQALQQNGSSVLSEDKSKRLNTILNTMSTIYSTGKVCNPDNPQECLLLEPGLNEIMANSLDYNERLWAWESWRSEVGKQLRPLYEEYVVLKNEMARANHYEDYGDYWRGDYEVNGVDGYDYSRGQLIEDVEHTFEEIKPLYEHLHAYVRAKLMNAYPSYISPIGCLPAHLLGDMWGRFWTNLYSLTVPFGQKPNIDVTDAMVDQAWDAQRIFKEAEKFFVSVGLPNMTPGFWENSMLTDPGNVQKAVCHPTAWDLGKGDFRILMCTKVTMDDFLTAHHEMGHIQYDMAYAAQPFLLRNGANEGFHEAVGEIMSLSAATPKHLKSIGLLSPDFQEDNETEINFLLKQALTIVGTLPFTYMLEKWRWMVFKGEIPKDQWMKKWWEMKREIVGVVEPVPHDETYCDPASLFHVSNDYSFIRYYTRTLYQFQFQEALCQAAKHEGPLHKCDISNSTEAGQKLFNMLRLGKSEPWTLALENVVGAKNMNVRPLLNYFEPLFTWLKDQNKNSFVGWSTDWSPYADQSIKVRISLKSALGDKAYEWNDNEMYLFRCSVAYAMRQYFLKVKNQMILFGEEDVRVANLKPRISFNFFVTAPKNVSDIIPRTEVEKAIRMSRSRINDAFRLNDNSLEFLGIQPTLGDKTHTCPPCPAPELLGGPSVFLFPPKPKDTLYITREPEVTCVVVDVSHEDPEVKFNWYVDGVEVHNAKTKPREEQYNSTYRVVSVLTVLHQDWLNGKEYKCKVSNKALPAPIEKTISKAKGQPREPQVYTLPPSRDELTKNQVSLTCLVKGFYPSDIAVEWESNGQPENNYKTTPPVLDSDGSFFLYSKLTVDKSRWQQGNVFSCSVMHEALHNHYTQKSLSLSPGK

SEQ ID NO: 61 - protein, 944 aa, synthetic construct
  REGION 1..944: note = ACE2 18-732 T92I Q325P S645C IgG4 T256D T307Q
QSTIEEQAKTFLDKFNHEAEDLFYQSSLASWNYNTNITEENVQNMNNAGDKWSAFLKEQSTLAQMYPLQEIQNLIVKLQLQALQQNGSSVLSEDKSKRLNTILNTMSTIYSTGKVCNPDNPQECLLLEPGLNEIMANSLDYNERLWAWESWRSEVGKQLRPLYEEYVVLKNEMARANHYEDYGDYWRGDYEVNGVDGYDYSRGQLIEDVEHTFEEIKPLYEHLHAYVRAKLMNAYPSYISPIGCLPAHLLGDMWGRFWTNLYSLTVPFGQKPNIDVTDAMVDQAWDAQRIFKEAEKFFVSVGLPNMTPGFWENSMLTDPGNVQKAVCHPTAWDLGKGDFRILMCTKVTMDDFLTAHHEMGHIQYDMAYAAQPFLLRNGANEGFHEAVGEIMSLSAATPKHLKSIGLLSPDFQEDNETEINFLLKQALTIVGTLPFTYMLEKWRWMVFKGEIPKDQWMKKWWEMKREIVGVVEPVPHDETYCDPASLFHVSNDYSFIRYYTRTLYQFQFQEALCQAAKHEGPLHKCDISNSTEAGQKLFNMLRLGKSEPWTLALENVVGAKNMNVRPLLNYFEPLFTWLKDQNKNSFVGWSTDWSPYADQSIKVRISLKSALGDKAYEWNDNEMYLFRCSVAYAMRQYFLKVKNQMILFGEEDVRVANLKPRISFNFFVTAPKNVSDIIPRTEVEKAIRMSRSRINDAFRLNDNSLEFLGIQPTLGESKYGPPCPPCPAPEFLGGPSVFLFPPKPKDTLMISRDPEVTCVVVDVSQEDPEVQFNWYVDGVEVHNAKTKPREEQFNSTYRVVSVLQVLHQDWLNGKEYKCKVSNKGLPSSIEKTISKAKGQPREPQVYTLPPSQEEMTKNQVSLTCLVKGFYPSDIAVEWESNGQPENNYKTTPPVLDSDGSFFLYSRLTVDKSRWQEGNVFSCSVMHEALHNHYTQKSLSLSLGK

SEQ ID NO: 62 - protein, 942 aa, synthetic construct
  REGION 1..942: note = ACE2 18-732 T92I Q325P S645C IgG1 T256D T307Q
QSTIEEQAKTFLDKFNHEAEDLFYQSSLASWNYNTNITEENVQNMNNAGDKWSAFLKEQSTLAQMYPLQEIQNLIVKLQLQALQQNGSSVLSEDKSKRLNTILNTMSTIYSTGKVCNPDNPQECLLLEPGLNEIMANSLDYNERLWAWESWRSEVGKQLRPLYEEYVVLKNEMARANHYEDYGDYWRGDYEVNGVDGYDYSRGQLIEDVEHTFEEIKPLYEHLHAYVRAKLMNAYPSYISPIGCLPAHLLGDMWGRFWTNLYSLTVPFGQKPNIDVTDAMVDQAWDAQRIFKEAEKFFVSVGLPNMTPGFWENSMLTDPGNVQKAVCHPTAWDLGKGDFRILMCTKVTMDDFLTAHHEMGHIQYDMAYAAQPFLLRNGANEGFHEAVGEIMSLSAATPKHLKSIGLLSPDFQEDNETEINFLLKQALTIVGTLPFTYMLEKWRWMVFKGEIPKDQWMKKWWEMKREIVGVVEPVPHDETYCDPASLFHVSNDYSFIRYYTRTLYQFQFQEALCQAAKHEGPLHKCDISNSTEAGQKLFNMLRLGKSEPWTLALENVVGAKNMNVRPLLNYFEPLFTWLKDQNKNSFVGWSTDWSPYADQSIKVRISLKSALGDKAYEWNDNEMYLFRCSVAYAMRQYFLKVKNQMILFGEEDVRVANLKPRISFNFFVTAPKNVSDIIPRTEVEKAIRMSRSRINDAFRLNDNSLEFLGIQPTLGDKTHTCPPCPAPELLGGPSVFLFPPKPKDTLMISRDPEVTCVVVDVSHEDPEVKFNWYVDGVEVHNAKTKPREEQYNSTYRVVSVLQVLHQDWLNGKEYKCKVSNKALPAPIEKTISKAKGQPREPQVYTLPPSRDELTKNQVSLTCLVKGFYPSDIAVEWESNGQPENNYKTTPPVLDSDGSFFLYSKLTVDKSRWQQGNVFSCSVMHEALHNHYTQKSLSLSPGK

SEQ ID NO: 63 - protein, 944 aa, synthetic construct
  REGION 1..715: note = ACE2 18-732 T27A T92I Q325P S645C IgG4 YTE
QSTIEEQAKAFLDKFNHEAEDLFYQSSLASWNYNTNITEENVQNMNNAGDKWSAFLKEQSTLAQMYPLQEIQNLIVKLQLQALQQNGSSVLSEDKSKRLNTILNTMSTIYSTGKVCNPDNPQECLLLEPGLNEIMANSLDYNERLWAWESWRSEVGKQLRPLYEEYVVLKNEMARANHYEDYGDYWRGDYEVNGVDGYDYSRGQLIEDVEHTFEEIKPLYEHLHAYVRAKLMNAYPSYISPIGCLPAHLLGDMWGRFWTNLYSLTVPFGQKPNIDVTDAMVDQAWDAQRIFKEAEKFFVSVGLPNMTPGFWENSMLTDPGNVQKAVCHPTAWDLGKGDFRILMCTKVTMDDFLTAHHEMGHIQYDMAYAAQPFLLRNGANEGFHEAVGEIMSLSAATPKHLKSIGLLSPDFQEDNETEINFLLKQALTIVGTLPFTYMLEKWRWMVFKGEIPKDQWMKKWWEMKREIVGVVEPVPHDETYCDPASLFHVSNDYSFIRYYTRTLYQFQFQEALCQAAKHEGPLHKCDISNSTEAGQKLFNMLRLGKSEPWTLALENVVGAKNMNVRPLLNYFEPLFTWLKDQNKNSFVGWSTDWSPYADQSIKVRISLKSALGDKAYEWNDNEMYLFRCSVAYAMRQYFLKVKNQMILFGEEDVRVANLKPRISFNFFVTAPKNVSDIIPRTEVEKAIRMSRSRINDAFRLNDNSLEFLGIQPTLGESKYGPPCPPCPAPEFLGGPSVFLFPPKPKDTLYITREPEVTCVVVDVSQEDPEVQFNWYVDGVEVHNAKTKPREEQFNSTYRVVSVLTVLHQDWLNGKEYKCKVSNKGLPSSIEKTISKAKGQPREPQVYTLPPSQEEMTKNQVSLTCLVKGFYPSDIAVEWESNGQPENNYKTTPPVLDSDGSFFLYSRLTVDKSRWQEGNVFSCSVMHEALHNHYTQKSLSLSLGK

SEQ ID NO: 64 - protein, 942 aa, synthetic construct
  REGION 1..723: note = ACE2 18-732 T27A T92I Q325P S645C IgG1 YTE
QSTIEEQAKAFLDKFNHEAEDLFYQSSLASWNYNTNITEENVQNMNNAGDKWSAFLKEQSTLAQMYPLQEIQNLIVKLQLQALQQNGSSVLSEDKSKRLNTILNTMSTIYSTGKVCNPDNPQECLLLEPGLNEIMANSLDYNERLWAWESWRSEVGKQLRPLYEEYVVLKNEMARANHYEDYGDYWRGDYEVNGVDGYDYSRGQLIEDVEHTFEEIKPLYEHLHAYVRAKLMNAYPSYISPIGCLPAHLLGDMWGRFWTNLYSLTVPFGQKPNIDVTDAMVDQAWDAQRIFKEAEKFFVSVGLPNMTPGFWENSMLTDPGNVQKAVCHPTAWDLGKGDFRILMCTKVTMDDFLTAHHEMGHIQYDMAYAAQPFLLRNGANEGFHEAVGEIMSLSAATPKHLKSIGLLSPDFQEDNETEINFLLKQALTIVGTLPFTYMLEKWRWMVFKGEIPKDQWMKKWWEMKREIVGVVEPVPHDETYCDPASLFHVSNDYSFIRYYTRTLYQFQFQEALCQAAKHEGPLHKCDISNSTEAGQKLFNMLRLGKSEPWTLALENVVGAKNMNVRPLLNYFEPLFTWLKDQNKNSFVGWSTDWSPYADQSIKVRISLKSALGDKAYEWNDNEMYLFRCSVAYAMRQYFLKVKNQMILFGEEDVRVANLKPRISFNFFVTAPKNVSDIIPRTEVEKAIRMSRSRINDAFRLNDNSLEFLGIQPTLGDKTHTCPPCPAPELLGGPSVFLFPPKPKDTLYITREPEVTCVVVDVSHEDPEVKFNWYVDGVEVHNAKTKPREEQYNSTYRVVSVLTVLHQDWLNGKEYKCKVSNKALPAPIEKTISKAKGQPREPQVYTLPPSRDELTKNQVSLTCLVKGFYPSDIAVEWESNGQPENNYKTTPPVLDSDGSFFLYSKLTVDKSRWQQGNVFSCSVMHEALHNHYTQKSLSLSPGK

SEQ ID NO: 65 - protein, 944 aa, synthetic construct
  REGION 1..944: note = ACE2 18-732 T27A T92I Q325P S645C IgG4 T256D T307Q
QSTIEEQAKAFLDKFNHEAEDLFYQSSLASWNYNTNITEENVQNMNNAGDKWSAFLKEQSTLAQMYPLQEIQNLIVKLQLQALQQNGSSVLSEDKSKRLNTILNTMSTIYSTGKVCNPDNPQECLLLEPGLNEIMANSLDYNERLWAWESWRSEVGKQLRPLYEEYVVLKNEMARANHYEDYGDYWRGDYEVNGVDGYDYSRGQLIEDVEHTFEEIKPLYEHLHAYVRAKLMNAYPSYISPIGCLPAHLLGDMWGRFWTNLYSLTVPFGQKPNIDVTDAMVDQAWDAQRIFKEAEKFFVSVGLPNMTPGFWENSMLTDPGNVQKAVCHPTAWDLGKGDFRILMCTKVTMDDFLTAHHEMGHIQYDMAYAAQPFLLRNGANEGFHEAVGEIMSLSAATPKHLKSIGLLSPDFQEDNETEINFLLKQALTIVGTLPFTYMLEKWRWMVFKGEIPKDQWMKKWWEMKREIVGVVEPVPHDETYCDPASLFHVSNDYSFIRYYTRTLYQFQFQEALCQAAKHEGPLHKCDISNSTEAGQKLFNMLRLGKSEPWTLALENVVGAKNMNVRPLLNYFEPLFTWLKDQNKNSFVGWSTDWSPYADQSIKVRISLKSALGDKAYEWNDNEMYLFRCSVAYAMRQYFLKVKNQMILFGEEDVRVANLKPRISFNFFVTAPKNVSDIIPRTEVEKAIRMSRSRINDAFRLNDNSLEFLGIQPTLGESKYGPPCPPCPAPEFLGGPSVFLFPPKPKDTLMISRDPEVTCVVVDVSQEDPEVQFNWYVDGVEVHNAKTKPREEQFNSTYRVVSVLQVLHQDWLNGKEYKCKVSNKGLPSSIEKTISKAKGQPREPQVYTLPPSQEEMTKNQVSLTCLVKGFYPSDIAVEWESNGQPENNYKTTPPVLDSDGSFFLYSRLTVDKSRWQEGNVFSCSVMHEALHNHYTQKSLSLSLGK

SEQ ID NO: 66 - protein, 942 aa, synthetic construct
  REGION 1..942: note = ACE2 18-732 T27A T92I Q325P S645C with IgG1 T256D T307Q
QSTIEEQAKAFLDKFNHEAEDLFYQSSLASWNYNTNITEENVQNMNNAGDKWSAFLKEQSTLAQMYPLQEIQNLIVKLQLQALQQNGSSVLSEDKSKRLNTILNTMSTIYSTGKVCNPDNPQECLLLEPGLNEIMANSLDYNERLWAWESWRSEVGKQLRPLYEEYVVLKNEMARANHYEDYGDYWRGDYEVNGVDGYDYSRGQLIEDVEHTFEEIKPLYEHLHAYVRAKLMNAYPSYISPIGCLPAHLLGDMWGRFWTNLYSLTVPFGQKPNIDVTDAMVDQAWDAQRIFKEAEKFFVSVGLPNMTPGFWENSMLTDPGNVQKAVCHPTAWDLGKGDFRILMCTKVTMDDFLTAHHEMGHIQYDMAYAAQPFLLRNGANEGFHEAVGEIMSLSAATPKHLKSIGLLSPDFQEDNETEINFLLKQALTIVGTLPFTYMLEKWRWMVFKGEIPKDQWMKKWWEMKREIVGVVEPVPHDETYCDPASLFHVSNDYSFIRYYTRTLYQFQFQEALCQAAKHEGPLHKCDISNSTEAGQKLFNMLRLGKSEPWTLALENVVGAKNMNVRPLLNYFEPLFTWLKDQNKNSFVGWSTDWSPYADQSIKVRISLKSALGDKAYEWNDNEMYLFRCSVAYAMRQYFLKVKNQMILFGEEDVRVANLKPRISFNFFVTAPKNVSDIIPRTEVEKAIRMSRSRINDAFRLNDNSLEFLGIQPTLGDKTHTCPPCPAPELLGGPSVFLFPPKPKDTLMISRDPEVTCVVVDVSHEDPEVKFNWYVDGVEVHNAKTKPREEQYNSTYRVVSVLQVLHQDWLNGKEYKCKVSNKALPAPIEKTISKAKGQPREPQVYTLPPSRDELTKNQVSLTCLVKGFYPSDIAVEWESNGQPENNYKTTPPVLDSDGSFFLYSKLTVDKSRWQQGNVFSCSVMHEALHNHYTQKSLSLSPGK

SEQ ID NO: 67 - protein, 805 aa, synthetic construct [sequence omitted]

SEQ ID NO: 68 - protein, 944 aa, synthetic construct
  REGION 1..944: note = ACE2 18-732 T27A IgG4 wt
QSTIEEQAKAFLDKFNHEAEDLFYQSSLASWNYNTNITEENVQNMNNAGDKWSAFLKEQSTLAQMYPLQEIQNLTVKLQLQALQQNGSSVLSEDKSKRLNTILNTMSTIYSTGKVCNPDNPQECLLLEPGLNEIMANSLDYNERLWAWESWRSEVGKQLRPLYEEYVVLKNEMARANHYEDYGDYWRGDYEVNGVDGYDYSRGQLIEDVEHTFEEIKPLYEHLHAYVRAKLMNAYPSYISPIGCLPAHLLGDMWGRFWTNLYSLTVPFGQKPNIDVTDAMVDQAWDAQRIFKEAEKFFVSVGLPNMTQGFWENSMLTDPGNVQKAVCHPTAWDLGKGDFRILMCTKVTMDDFLTAHHEMGHIQYDMAYAAQPFLLRNGANEGFHEAVGEIMSLSAATPKHLKSIGLLSPDFQEDNETEINFLLKQALTIVGTLPFTYMLEKWRWMVFKGEIPKDQWMKKWWEMKREIVGVVEPVPHDETYCDPASLFHVSNDYSFIRYYTRTLYQFQFQEALCQAAKHEGPLHKCDISNSTEAGQKLFNMLRLGKSEPWTLALENVVGAKNMNVRPLLNYFEPLFTWLKDQNKNSFVGWSTDWSPYADQSIKVRISLKSALGDKAYEWNDNEMYLFRSSVAYAMRQYFLKVKNQMILFGEEDVRVANLKPRISFNFFVTAPKNVSDIIPRTEVEKAIRMSRSRINDAFRLNDNSLEFLGIQPTLGESKYGPPCPPCPAPEFLGGPSVFLFPPKPKDTLMISRTPEVTCVVVDVSQEDPEVQFNWYVDGVEVHNAKTKPREEQFNSTYRVVSVLTVLHQDWLNGKEYKCKVSNKGLPSSIEKTISKAKGQPREPQVYTLPPSQEEMTKNQVSLTCLVKGFYPSDIAVEWESNGQPENNYKTTPPVLDSDGSFFLYSRLTVDKSRWQEGNVFSCSVMHEALHNHYTQKSLSLSLGK

SEQ ID NO: 69 - protein, 942 aa, synthetic construct
  REGION 1..942: note = ACE2 18-732 T27A IgG1 wt
QSTIEEQAKAFLDKFNHEAEDLFYQSSLASWNYNTNITEENVQNMNNAGDKWSAFLKEQSTLAQMYPLQEIQNLTVKLQLQALQQNGSSVLSEDKSKRLNTILNTMSTIYSTGKVCNPDNPQECLLLEPGLNEIMANSLDYNERLWAWESWRSEVGKQLRPLYEEYVVLKNEMARANHYEDYGDYWRGDYEVNGVDGYDYSRGQLIEDVEHTFEEIKPLYEHLHAYVRAKLMNAYPSYISPIGCLPAHLLGDMWGRFWTNLYSLTVPFGQKPNIDVTDAMVDQAWDAQRIFKEAEKFFVSVGLPNMTQGFWENSMLTDPGNVQKAVCHPTAWDLGKGDFRILMCTKVTMDDFLTAHHEMGHIQYDMAYAAQPFLLRNGANEGFHEAVGEIMSLSAATPKHLKSIGLLSPDFQEDNETEINFLLKQALTIVGTLPFTYMLEKWRWMVFKGEIPKDQWMKKWWEMKREIVGVVEPVPHDETYCDPASLFHVSNDYSFIRYYTRTLYQFQFQEALCQAAKHEGPLHKCDISNSTEAGQKLFNMLRLGKSEPWTLALENVVGAKNMNVRPLLNYFEPLFTWLKDQNKNSFVGWSTDWSPYADQSIKVRISLKSALGDKAYEWNDNEMYLFRSSVAYAMRQYFLKVKNQMILFGEEDVRVANLKPRISFNFFVTAPKNVSDIIPRTEVEKAIRMSRSRINDAFRLNDNSLEFLGIQPTLGDKTHTCPPCPAPELLGGPSVFLFPPKPKDTLMISRTPEVTCVVVDVSHEDPEVKFNWYVDGVEVHNAKTKPREEQYNSTYRVVSVLTVLHQDWLNGKEYKCKVSNKALPAPIEKTISKAKGQPREPQVYTLPPSRDELTKNQVSLTCLVKGFYPSDIAVEWESNGQPENNYKTTPPVLDSDGSFFLYSKLTVDKSRWQQGNVFSCSVMHEALHNHYTQKSLSLSPGK

SEQ ID NO: 70 - protein, 944 aa, synthetic construct
  REGION 1..944: note = ACE2 18-732 T92I IgG4 wt
QSTIEEQAKTFLDKFNHEAEDLFYQSSLASWNYNTNITEENVQNMNNAGDKWSAFLKEQSTLAQMYPLQEIQNLIVKLQLQALQQNGSSVLSEDKSKRLNTILNTMSTIYSTGKVCNPDNPQECLLLEPGLNEIMANSLDYNERLWAWESWRSEVGKQLRPLYEEYVVLKNEMARANHYEDYGDYWRGDYEVNGVDGYDYSRGQLIEDVEHTFEEIKPLYEHLHAYVRAKLMNAYPSYISPIGCLPAHLLGDMWGRFWTNLYSLTVPFGQKPNIDVTDAMVDQAWDAQRIFKEAEKFFVSVGLPNMTQGFWENSMLTDPGNVQKAVCHPTAWDLGKGDFRILMCTKVTMDDFLTAHHEMGHIQYDMAYAAQPFLLRNGANEGFHEAVGEIMSLSAATPKHLKSIGLLSPDFQEDNETEINFLLKQALTIVGTLPFTYMLEKWRWMVFKGEIPKDQWMKKWWEMKREIVGVVEPVPHDETYCDPASLFHVSNDYSFIRYYTRTLYQFQFQEALCQAAKHEGPLHKCDISNSTEAGQKLFNMLRLGKSEPWTLALENVVGAKNMNVRPLLNYFEPLFTWLKDQNKNSFVGWSTDWSPYADQSIKVRISLKSALGDKAYEWNDNEMYLFRSSVAYAMRQYFLKVKNQMILFGEEDVRVANLKPRISFNFFVTAPKNVSDIIPRTEVEKAIRMSRSRINDAFRLNDNSLEFLGIQPTLGESKYGPPCPPCPAPEFLGGPSVFLFPPKPKDTLMISRTPEVTCVVVDVSQEDPEVQFNWYVDGVEVHNAKTKPREEQFNSTYRVVSVLTVLHQDWLNGKEYKCKVSNKGLPSSIEKTISKAKGQPREPQVYTLPPSQEEMTKNQVSLTCLVKGFYPSDIAVEWESNGQPENNYKTTPPVLDSDGSFFLYSRLTVDKSRWQEGNVFSCSVMHEALHNHYTQKSLSLSLGK

SEQ ID NO: 71 - protein, 942 aa, synthetic construct
  REGION 1..942: note = ACE2 18-732 T92I IgG1 wt
QSTIEEQAKTFLDKFNHEAEDLFYQSSLASWNYNTNITEENVQNMNNAGDKWSAFLKEQSTLAQMYPLQEIQNLIVKLQLQALQQNGSSVLSEDKSKRLNTILNTMSTIYSTGKVCNPDNPQECLLLEPGLNEIMANSLDYNERLWAWESWRSEVGKQLRPLYEEYVVLKNEMARANHYEDYGDYWRGDYEVNGVDGYDYSRGQLIEDVEHTFEEIKPLYEHLHAYVRAKLMNAYPSYISPIGCLPAHLLGDMWGRFWTNLYSLTVPFGQKPNIDVTDAMVDQAWDAQRIFKEAEKFFVSVGLPNMTQGFWENSMLTDPGNVQKAVCHPTAWDLGKGDFRILMCTKVTMDDFLTAHHEMGHIQYDMAYAAQPFLLRNGANEGFHEAVGEIMSLSAATPKHLKSIGLLSPDFQEDNETEINFLLKQALTIVGTLPFTYMLEKWRWMVFKGEIPKDQWMKKWWEMKREIVGVVEPVPHDETYCDPASLFHVSNDYSFIRYYTRTLYQFQFQEALCQAAKHEGPLHKCDISNSTEAGQKLFNMLRLGKSEPWTLALENVVGAKNMNVRPLLNYFEPLFTWLKDQNKNSFVGWSTDWSPYADQSIKVRISLKSALGDKAYEWNDNEMYLFRSSVAYAMRQYFLKVKNQMILFGEEDVRVANLKPRISFNFFVTAPKNVSDIIPRTEVEKAIRMSRSRINDAFRLNDNSLEFLGIQPTLGDKTHTCPPCPAPELLGGPSVFLFPPKPKDTLMISRTPEVTCVVVDVSHEDPEVKFNWYVDGVEVHNAKTKPREEQYNSTYRVVSVLTVLHQDWLNGKEYKCKVSNKALPAPIEKTISKAKGQPREPQVYTLPPSRDELTKNQVSLTCLVKGFYPSDIAVEWESNGQPENNYKTTPPVLDSDGSFFLYSKLTVDKSRWQQGNVFSCSVMHEALHNHYTQKSLSLSPGK

SEQ ID NO: 72 - protein, 944 aa, synthetic construct
  REGION 1..944: note = ACE2 18-732 Q325P IgG4 wt
QSTIEEQAKTFLDKFNHEAEDLFYQSSLASWNYNTNITEENVQNMNNAGDKWSAFLKEQSTLAQMYPLQEIQNLTVKLQLQALQQNGSSVLSEDKSKRLNTILNTMSTIYSTGKVCNPDNPQECLLLEPGLNEIMANSLDYNERLWAWESWRSEVGKQLRPLYEEYVVLKNEMARANHYEDYGDYWRGDYEVNGVDGYDYSRGQLIEDVEHTFEEIKPLYEHLHAYVRAKLMNAYPSYISPIGCLPAHLLGDMWGRFWTNLYSLTVPFGQKPNIDVTDAMVDQAWDAQRIFKEAEKFFVSVGLPNMTPGFWENSMLTDPGNVQKAVCHPTAWDLGKGDFRILMCTKVTMDDFLTAHHEMGHIQYDMAYAAQPFLLRNGANEGFHEAVGEIMSLSAATPKHLKSIGLLSPDFQEDNETEINFLLKQALTIVGTLPFTYMLEKWRWMVFKGEIPKDQWMKKWWEMKREIVGVVEPVPHDETYCDPASLFHVSNDYSFIRYYTRTLYQFQFQEALCQAAKHEGPLHKCDISNSTEAGQKLFNMLRLGKSEPWTLALENVVGAKNMNVRPLLNYFEPLFTWLKDQNKNSFVGWSTDWSPYADQSIKVRISLKSALGDKAYEWNDNEMYLFRSSVAYAMRQYFLKVKNQMILFGEEDVRVANLKPRISFNFFVTAPKNVSDIIPRTEVEKAIRMSRSRINDAFRLNDNSLEFLGIQPTLGESKYGPPCPPCPAPEFLGGPSVFLFPPKPKDTLMISRTPEVTCVVVDVSQEDPEVQFNWYVDGVEVHNAKTKPREEQFNSTYRVVSVLTVLHQDWLNGKEYKCKVSNKGLPSSIEKTISKAKGQPREPQVYTLPPSQEEMTKNQVSLTCLVKGFYPSDIAVEWESNGQPENNYKTTPPVLDSDGSFFLYSRLTVDKSRWQEGNVFSCSVMHEALHNHYTQKSLSLSLGK

SEQ ID NO: 73 - protein, 942 aa, synthetic construct
  REGION 1..942: note = ACE2 18-732 Q325P IgG1 wt
QSTIEEQAKTFLDKFNHEAEDLFYQSSLASWNYNTNITEENVQNMNNAGDKWSAFLKEQSTLAQMYPLQEIQNLTVKLQLQALQQNGSSVLSEDKSKRLNTILNTMSTIYSTGKVCNPDNPQECLLLEPGLNEIMANSLDYNERLWAWESWRSEVGKQLRPLYEEYVVLKNEMARANHYEDYGDYWRGDYEVNGVDGYDYSRGQLIEDVEHTFEEIKPLYEHLHAYVRAKLMNAYPSYISPIGCLPAHLLGDMWGRFWTNLYSLTVPFGQKPNIDVTDAMVDQAWDAQRIFKEAEKFFVSVGLPNMTPGFWENSMLTDPGNVQKAVCHPTAWDLGKGDFRILMCTKVTMDDFLTAHHEMGHIQYDMAYAAQPFLLRNGANEGFHEAVGEIMSLSAATPKHLKSIGLLSPDFQEDNETEINFLLKQALTIVGTLPFTYMLEKWRWMVFKGEIPKDQWMKKWWEMKREIVGVVEPVPHDETYCDPASLFHVSNDYSFIRYYTRTLYQFQFQEALCQAAKHEGPLHKCDISNSTEAGQKLFNMLRLGKSEPWTLALENVVGAKNMNVRPLLNYFEPLFTWLKDQNKNSFVGWSTDWSPYADQSIKVRISLKSALGDKAYEWNDNEMYLFRSSVAYAMRQYFLKVKNQMILFGEEDVRVANLKPRISFNFFVTAPKNVSDIIPRTEVEKAIRMSRSRINDAFRLNDNSLEFLGIQPTLGDKTHTCPPCPAPELLGGPSVFLFPPKPKDTLMISRTPEVTCVVVDVSHEDPEVKFNWYVDGVEVHNAKTKPREEQYNSTYRVVSVLTVLHQDWLNGKEYKCKVSNKALPAPIEKTISKAKGQPREPQVYTLPPSRDELTKNQVSLTCLVKGFYPSDIAVEWESNGQPENNYKTTPPVLDSDGSFFLYSKLTVDKSRWQQGNVFSCSVMHEALHNHYTQKSLSLSPGK

SEQ ID NO: 74 - protein, 944 aa, synthetic construct
  REGION 1..944: note = ACE2 18-732 T27A S645C IgG4 wt
QSTIEEQAKAFLDKFNHEAEDLFYQSSLASWNYNTNITEENVQNMNNAGDKWSAFLKEQSTLAQMYPLQEIQNLTVKLQLQALQQNGSSVLSEDKSKRLNTILNTMSTIYSTGKVCNPDNPQECLLLEPGLNEIMANSLDYNERLWAWESWRSEVGKQLRPLYEEYVVLKNEMARANHYEDYGDYWRGDYEVNGVDGYDYSRGQLIEDVEHTFEEIKPLYEHLHAYVRAKLMNAYPSYISPIGCLPAHLLGDMWGRFWTNLYSLTVPFGQKPNIDVTDAMVDQAWDAQRIFKEAEKFFVSVGLPNMTQGFWENSMLTDPGNVQKAVCHPTAWDLGKGDFRILMCTKVTMDDFLTAHHEMGHIQYDMAYAAQPFLLRNGANEGFHEAVGEIMSLSAATPKHLKSIGLLSPDFQEDNETEINFLLKQALTIVGTLPFTYMLEKWRWMVFKGEIPKDQWMKKWWEMKREIVGVVEPVPHDETYCDPASLFHVSNDYSFIRYYTRTLYQFQFQEALCQAAKHEGPLHKCDISNSTEAGQKLFNMLRLGKSEPWTLALENVVGAKNMNVRPLLNYFEPLFTWLKDQNKNSFVGWSTDWSPYADQSIKVRISLKSALGDKAYEWNDNEMYLFRCSVAYAMRQYFLKVKNQMILFGEEDVRVANLKPRISFNFFVTAPKNVSDIIPRTEVEKAIRMSRSRINDAFRLNDNSLEFLGIQPTLGESKYGPPCPPCPAPEFLGGPSVFLFPPKPKDTLMISRTPEVTCVVVDVSQEDPEVQFNWYVDGVEVHNAKTKPREEQFNSTYRVVSVLTVLHQDWLNGKEYKCKVSNKGLPSSIEKTISKAKGQPREPQVYTLPPSQEEMTKNQVSLTCLVKGFYPSDIAVEWESNGQPENNYKTTPPVLDSDGSFFLYSRLTVDKSRWQEGNVFSCSVMHEALHNHYTQKSLSLSLGK

SEQ ID NO: 75 - protein, 942 aa, synthetic construct
  REGION 1..942: note = ACE2 18-732 T27A S645C IgG1 wt
QSTIEEQAKAFLDKFNHEAEDLFYQSSLASWNYNTNITEENVQNMNNAGDKWSAFLKEQSTLAQMYPLQEIQNLTVKLQLQALQQNGSSVLSEDKSKRLNTILNTMSTIYSTGKVCNPDNPQECLLLEPGLNEIMANSLDYNERLWAWESWRSEVGKQLRPLYEEYVVLKNEMARANHYEDYGDYWRGDYEVNGVDGYDYSRGQLIEDVEHTFEEIKPLYEHLHAYVRAKLMNAYPSYISPIGCLPAHLLGDMWGRFWTNLYSLTVPFGQKPNIDVTDAMVDQAWDAQRIFKEAEKFFVSVGLPNMTQGFWENSMLTDPGNVQKAVCHPTAWDLGKGDFRILMCTKVTMDDFLTAHHEMGHIQYDMAYAAQPFLLRNGANEGFHEAVGEIMSLSAATPKHLKSIGLLSPDFQEDNETEINFLLKQALTIVGTLPFTYMLEKWRWMVFKGEIPKDQWMKKWWEMKREIVGVVEPVPHDETYCDPASLFHVSNDYSFIRYYTRTLYQFQFQEALCQAAKHEGPLHKCDISNSTEAGQKLFNMLRLGKSEPWTLALENVVGAKNMNVRPLLNYFEPLFTWLKDQNKNSFVGWSTDWSPYADQSIKVRISLKSALGDKAYEWNDNEMYLFRCSVAYAMRQYFLKVKNQMILFGEEDVRVANLKPRISFNFFVTAPKNVSDIIPRTEVEKAIRMSRSRINDAFRLNDNSLEFLGIQPTLGDKTHTCPPCPAPELLGGPSVFLFPPKPKDTLMISRTPEVTCVVVDVSHEDPEVKFNWYVDGVEVHNAKTKPREEQYNSTYRVVSVLTVLHQDWLNGKEYKCKVSNKALPAPIEKTISKAKGQPREPQVYTLPPSRDELTKNQVSLTCLVKGFYPSDIAVEWESNGQPENNYKTTPPVLDSDGSFFLYSKLTVDKSRWQQGNVFSCSVMHEALHNHYTQKSLSLSPGK

SEQ ID NO: 76 - protein, 944 aa, synthetic construct
  REGION 1..944: note = ACE2 18-732 T92I S645C IgG4 wt
QSTIEEQAKTFLDKFNHEAEDLFYQSSLASWNYNTNITEENVQNMNNAGDKWSAFLKEQSTLAQMYPLQEIQNLIVKLQLQALQQNGSSVLSEDKSKRLNTILNTMSTIYSTGKVCNPDNPQECLLLEPGLNEIMANSLDYNERLWAWESWRSEVGKQLRPLYEEYVVLKNEMARANHYEDYGDYWRGDYEVNGVDGYDYSRGQLIEDVEHTFEEIKPLYEHLHAYVRAKLMNAYPSYISPIGCLPAHLLGDMWGRFWTNLYSLTVPFGQKPNIDVTDAMVDQAWDAQRIFKEAEKFFVSVGLPNMTQGFWENSMLTDPGNVQKAVCHPTAWDLGKGDFRILMCTKVTMDDFLTAHHEMGHIQYDMAYAAQPFLLRNGANEGFHEAVGEIMSLSAATPKHLKSIGLLSPDFQEDNETEINFLLKQALTIVGTLPFTYMLEKWRWMVFKGEIPKDQWMKKWWEMKREIVGVVEPVPHDETYCDPASLFHVSNDYSFIRYYTRTLYQFQFQEALCQAAKHEGPLHKCDISNSTEAGQKLFNMLRLGKSEPWTLALENVVGAKNMNVRPLLNYFEPLFTWLKDQNKNSFVGWSTDWSPYADQSIKVRISLKSALGDKAYEWNDNEMYLFRCSVAYAMRQYFLKVKNQMILFGEEDVRVANLKPRISFNFFVTAPKNVSDIIPRTEVEKAIRMSRSRINDAFRLNDNSLEFLGIQPTLGESKYGPPCPPCPAPEFLGGPSVFLFPPKPKDTLMISRTPEVTCVVVDVSQEDPEVQFNWYVDGVEVHNAKTKPREEQFNSTYRVVSVLTVLHQDWLNGKEYKCKVSNKGLPSSIEKTISKAKGQPREPQVYTLPPSQEEMTKNQVSLTCLVKGFYPSDIAVEWESNGQPENNYKTTPPVLDSDGSFFLYSRLTVDKSRWQEGNVFSCSVMHEALHNHYTQKSLSLSLGK

SEQ ID NO: 77 - protein, 942 aa, synthetic construct
  REGION 1..942: note = ACE2 18-732 T92I S645C IgG1 wt
QSTIEEQAKTFLDKFNHEAEDLFYQSSLASWNYNTNITEENVQNMNNAGDKWSAFLKEQSTLAQMYPLQEIQNLIVKLQLQALQQNGSSVLSEDKSKRLNTILNTMSTIYSTGKVCNPDNPQECLLLEPGLNEIMANSLDYNERLWAWESWRSEVGKQLRPLYEEYVVLKNEMARANHYEDYGDYWRGDYEVNGVDGYDYSRGQLIEDVEHTFEEIKPLYEHLHAYVRAKLMNAYPSYISPIGCLPAHLLGDMWGRFWTNLYSLTVPFGQKPNIDVTDAMVDQAWDAQRIFKEAEKFFVSVGLPNMTQGFWENSMLTDPGNVQKAVCHPTAWDLGKGDFRILMCTKVTMDDFLTAHHEMGHIQYDMAYAAQPFLLRNGANEGFHEAVGEIMSLSAATPKHLKSIGLLSPDFQEDNETEINFLLKQALTIVGTLPFTYMLEKWRWMVFKGEIPKDQWMKKWWEMKREIVGVVEPVPHDETYCDPASLFHVSNDYSFIRYYTRTLYQFQFQEALCQAAKHEGPLHKCDISNSTEAGQKLFNMLRLGKSEPWTLALENVVGAKNMNVRPLLNYFEPLFTWLKDQNKNSFVGWSTDWSPYADQSIKVRISLKSALGDKAYEWNDNEMYLFRCSVAYAMRQYFLKVKNQMILFGEEDVRVANLKPRISFNFFVTAPKNVSDIIPRTEVEKAIRMSRSRINDAFRLNDNSLEFLGIQPTLGDKTHTCPPCPAPELLGGPSVFLFPPKPKDTLMISRTPEVTCVVVDVSHEDPEVKFNWYVDGVEVHNAKTKPREEQYNSTYRVVSVLTVLHQDWLNGKEYKCKVSNKALPAPIEKTISKAKGQPREPQVYTLPPSRDELTKNQVSLTCLVKGFYPSDIAVEWESNGQPENNYKTTPPVLDSDGSFFLYSKLTVDKSRWQQGNVFSCSVMHEALHNHYTQKSLSLSPGK

SEQ ID NO: 78 - protein, 944 aa, synthetic construct
  REGION 1..944: note = ACE2 18-732 Q325P S645C IgG4 wt
QSTIEEQAKTFLDKFNHEAEDLFYQSSLASWNYNTNITEENVQNMNNAGDKWSAFLKEQSTLAQMYPLQEIQNLTVKLQLQALQQNGSSVLSEDKSKRLNTILNTMSTIYSTGKVCNPDNPQECLLLEPGLNEIMANSLDYNERLWAWESWRSEVGKQLRPLYEEYVVLKNEMARANHYEDYGDYWRGDYEVNGVDGYDYSRGQLIEDVEHTFEEIKPLYEHLHAYVRAKLMNAYPSYISPIGCLPAHLLGDMWGRFWTNLYSLTVPFGQKPNIDVTDAMVDQAWDAQRIFKEAEKFFVSVGLPNMTPGFWENSMLTDPGNVQKAVCHPTAWDLGKGDFRILMCTKVTMDDFLTAHHEMGHIQYDMAYAAQPFLLRNGANEGFHEAVGEIMSLSAATPKHLKSIGLLSPDFQEDNETEINFLLKQALTIVGTLPFTYMLEKWRWMVFKGEIPKDQWMKKWWEMKREIVGVVEPVPHDETYCDPASLFHVSNDYSFIRYYTRTLYQFQFQEALCQAAKHEGPLHKCDISNSTEAGQKLFNMLRLGKSEPWTLALENVVGAKNMNVRPLLNYFEPLFTWLKDQNKNSFVGWSTDWSPYADQSIKVRISLKSALGDKAYEWNDNEMYLFRCSVAYAMRQYFLKVKNQMILFGEEDVRVANLKPRISFNFFVTAPKNVSDIIPRTEVEKAIRMSRSRINDAFRLNDNSLEFLGIQPTLGESKYGPPCPPCPAPEFLGGPSVFLFPPKPKDTLMISRTPEVTCVVVDVSQEDPEVQFNWYVDGVEVHNAKTKPREEQFNSTYRVVSVLTVLHQDWLNGKEYKCKVSNKGLPSSIEKTISKAKGQPREPQVYTLPPSQEEMTKNQVSLTCLVKGFYPSDIAVEWESNGQPENNYKTTPPVLDSDGSFFLYSRLTVDKSRWQEGNVFSCSVMHEALHNHYTQKSLSLSLGK

SEQ ID NO: 79 - protein, 942 aa, synthetic construct
  REGION 1..942: note = ACE2 18-732 Q325P S645C IgG1 wt
QSTIEEQAKTFLDKFNHEAEDLFYQSSLASWNYNTNITEENVQNMNNAGDKWSAFLKEQSTLAQMYPLQEIQNLTVKLQLQALQQNGSSVLSEDKSKRLNTILNTMSTIYSTGKVCNPDNPQECLLLEPGLNEIMANSLDYNERLWAWESWRSEVGKQLRPLYEEYVVLKNEMARANHYEDYGDYWRGDYEVNGVDGYDYSRGQLIEDVEHTFEEIKPLYEHLHAYVRAKLMNAYPSYISPIGCLPAHLLGDMWGRFWTNLYSLTVPFGQKPNIDVTDAMVDQAWDAQRIFKEAEKFFVSVGLPNMTPGFWENSMLTDPGNVQKAVCHPTAWDLGKGDFRILMCTKVTMDDFLTAHHEMGHIQYDMAYAAQPFLLRNGANEGFHEAVGEIMSLSAATPKHLKSIGLLSPDFQEDNETEINFLLKQALTIVGTLPFTYMLEKWRWMVFKGEIPKDQWMKKWWEMKREIVGVVEPVPHDETYCDPASLFHVSNDYSFIRYYTRTLYQFQFQEALCQAAKHEGPLHKCDISNSTEAGQKLFNMLRLGKSEPWTLALENVVGAKNMNVRPLLNYFEPLFTWLKDQNKNSFVGWSTDWSPYADQSIKVRISLKSALGDKAYEWNDNEMYLFRCSVAYAMRQYFLKVKNQMILFGEEDVRVANLKPRISFNFFVTAPKNVSDIIPRTEVEKAIRMSRSRINDAFRLNDNSLEFLGIQPTLGDKTHTCPPCPAPELLGGPSVFLFPPKPKDTLMISRTPEVTCVVVDVSHEDPEVKFNWYVDGVEVHNAKTKPREEQYNSTYRVVSVLTVLHQDWLNGKEYKCKVSNKALPAPIEKTISKAKGQPREPQVYTLPPSRDELTKNQVSLTCLVKGFYPSDIAVEWESNGQPENNYKTTPPVLDSDGSFFLYSKLTVDKSRWQQGNVFSCSVMHEALHNHYTQKSLSLSPGK

SEQ ID NO: 80 - protein, 944 aa, synthetic construct
  REGION 1..944: note = ACE2 18-732 T27A T92I S645C IgG4 wt
QSTIEEQAKAFLDKFNHEAEDLFYQSSLASWNYNTNITEENVQNMNNAGDKWSAFLKEQSTLAQMYPLQEIQNLIVKLQLQALQQNGSSVLSEDKSKRLNTILNTMSTIYSTGKVCNPDNPQECLLLEPGLNEIMANSLDYNERLWAWESWRSEVGKQLRPLYEEYVVLKNEMARANHYEDYGDYWRGDYEVNGVDGYDYSRGQLIEDVEHTFEEIKPLYEHLHAYVRAKLMNAYPSYISPIGCLPAHLLGDMWGRFWTNLYSLTVPFGQKPNIDVTDAMVDQAWDAQRIFKEAEKFFVSVGLPNMTQGFWENSMLTDPGNVQKAVCHPTAWDLGKGDFRILMCTKVTMDDFLTAHHEMGHIQYDMAYAAQPFLLRNGANEGFHEAVGEIMSLSAATPKHLKSIGLLSPDFQEDNETEINFLLKQALTIVGTLPFTYMLEKWRWMVFKGEIPKDQWMKKWWEMKREIVGVVEPVPHDETYCDPASLFHVSNDYSFIRYYTRTLYQFQFQEALCQAAKHEGPLHKCDISNSTEAGQKLFNMLRLGKSEPWTLALENVVGAKNMNVRPLLNYFEPLFTWLKDQNKNSFVGWSTDWSPYADQSIKVRISLKSALGDKAYEWNDNEMYLFRCSVAYAMRQYFLKVKNQMILFGEEDVRVANLKPRISFNFFVTAPKNVSDIIPRTEVEKAIRMSRSRINDAFRLNDNSLEFLGIQPTLGESKYGPPCPPCPAPEFLGGPSVFLFPPKPKDTLMISRTPEVTCVVVDVSQEDPEVQFNWYVDGVEVHNAKTKPREEQFNSTYRVVSVLTVLHQDWLNGKEYKCKVSNKGLPSSIEKTISKAKGQPREPQVYTLPPSQEEMTKNQVSLTCLVKGFYPSDIAVEWESNGQPENNYKTTPPVLDSDGSFFLYSRLTVDKSRWQEGNVFSCSVMHEALHNHYTQKSLSLSLGK

SEQ ID NO: 81 - protein, 942 aa, synthetic construct
  REGION 1..942: note = ACE2 18-732 T27A T92I S645C IgG1 wt
QSTIEEQAKAFLDKFNHEAEDLFYQSSLASWNYNTNITEENVQNMNNAGDKWSAFLKEQSTLAQMYPLQEIQNLIVKLQLQALQQNGSSVLSEDKSKRLNTILNTMSTIYSTGKVCNPDNPQECLLLEPGLNEIMANSLDYNERLWAWESWRSEVGKQLRPLYEEYVVLKNEMARANHYEDYGDYWRGDYEVNGVDGYDYSRGQLIEDVEHTFEEIKPLYEHLHAYVRAKLMNAYPSYISPIGCLPAHLLGDMWGRFWTNLYSLTVPFGQKPNIDVTDAMVDQAWDAQRIFKEAEKFFVSVGLPNMTQGFWENSMLTDPGNVQKAVCHPTAWDLGKGDFRILMCTKVTMDDFLTAHHEMGHIQYDMAYAAQPFLLRNGANEGFHEAVGEIMSLSAATPKHLKSIGLLSPDFQEDNETEINFLLKQALTIVGTLPFTYMLEKWRWMVFKGEIPKDQWMKKWWEMKREIVGVVEPVPHDETYCDPASLFHVSNDYSFIRYYTRTLYQFQFQEALCQAAKHEGPLHKCDISNSTEAGQKLFNMLRLGKSEPWTLALENVVGAKNMNVRPLLNYFEPLFTWLKDQNKNSFVGWSTDWSPYADQSIKVRISLKSALGDKAYEWNDNEMYLFRCSVAYAMRQYFLKVKNQMILFGEEDVRVANLKPRISFNFFVTAPKNVSDIIPRTEVEKAIRMSRSRINDAFRLNDNSLEFLGIQPTLGDKTHTCPPCPAPELLGGPSVFLFPPKPKDTLMISRTPEVTCVVVDVSHEDPEVKFNWYVDGVEVHNAKTKPREEQYNSTYRVVSVLTVLHQDWLNGKEYKCKVSNKALPAPIEKTISKAKGQPREPQVYTLPPSRDELTKNQVSLTCLVKGFYPSDIAVEWESNGQPENNYKTTPPVLDSDGSFFLYSKLTVDKSRWQQGNVFSCSVMHEALHNHYTQKSLSLSPGK

SEQ ID NO: 82 - protein, 944 aa, synthetic construct
  REGION 1..944: note = ACE2 18-732 T27A Q325P S645C IgG4 wt
QSTIEEQAKAFLDKFNHEAEDLFYQSSLASWNYNTNITEENVQNMNNAGDKWSAFLKEQSTLAQMYPLQEIQNLTVKLQLQALQQNGSSVLSEDKSKRLNTILNTMSTIYSTGKVCNPDNPQECLLLEPGLNEIMANSLDYNERLWAWESWRSEVGKQLRPLYEEYVVLKNEMARANHYEDYGDYWRGDYEVNGVDGYDYSRGQLIEDVEHTFEEIKPLYEHLHAYVRAKLMNAYPSYISPIGCLPAHLLGDMWGRFWTNLYSLTVPFGQKPNIDVTDAMVDQAWDAQRIFKEAEKFFVSVGLPNMTPGFWENSMLTDPGNVQKAVCHPTAWDLGKGDFRILMCTKVTMDDFLTAHHEMGHIQYDMAYAAQPFLLRNGANEGFHEAVGEIMSLSAATPKHLKSIGLLSPDFQEDNETEINFLLKQALTIVGTLPFTYMLEKWRWMVFKGEIPKDQWMKKWWEMKREIVGVVEPVPHDETYCDPASLFHVSNDYSFIRYYTRTLYQFQFQEALCQAAKHEGPLHKCDISNSTEAGQKLFNMLRLGKSEPWTLALENVVGAKNMNVRPLLNYFEPLFTWLKDQNKNSFVGWSTDWSPYADQSIKVRISLKSALGDKAYEWNDNEMYLFRCSVAYAMRQYFLKVKNQMILFGEEDVRVANLKPRISFNFFVTAPKNVSDIIPRTEVEKAIRMSRSRINDAFRLNDNSLEFLGIQPTLGESKYGPPCPPCPAPEFLGGPSVFLFPPKPKDTLMISRTPEVTCVVVDVSQEDPEVQFNWYVDGVEVHNAKTKPREEQFNSTYRVVSVLTVLHQDWLNGKEYKCKVSNKGLPSSIEKTISKAKGQPREPQVYTLPPSQEEMTKNQVSLTCLVKGFYPSDIAVEWESNGQPENNYKTTPPVLDSDGSFFLYSRLTVDKSRWQEGNVFSCSVMHEALHNHYTQKSLSLSLGK

SEQ ID NO: 83 - protein, 942 aa, synthetic construct
  REGION 1..942: note = ACE2 18-732 T27A Q325P S645C IgG1 wt
QSTIEEQAKAFLDKFNHEAEDLFYQSSLASWNYNTNITEENVQNMNNAGDKWSAFLKEQSTLAQMYPLQEIQNLTVKLQLQALQQNGSSVLSEDKSKRLNTILNTMSTIYSTGKVCNPDNPQECLLLEPGLNEIMANSLDYNERLWAWESWRSEVGKQLRPLYEEYVVLKNEMARANHYEDYGDYWRGDYEVNGVDGYDYSRGQLIEDVEHTFEEIKPLYEHLHAYVRAKLMNAYPSYISPIGCLPAHLLGDMWGRFWTNLYSLTVPFGQKPNIDVTDAMVDQAWDAQRIFKEAEKFFVSVGLPNMTPGFWENSMLTDPGNVQKAVCHPTAWDLGKGDFRILMCTKVTMDDFLTAHHEMGHIQYDMAYAAQPFLLRNGANEGFHEAVGEIMSLSAATPKHLKSIGLLSPDFQEDNETEINFLLKQALTIVGTLPFTYMLEKWRWMVFKGEIPKDQWMKKWWEMKREIVGVVEPVPHDETYCDPASLFHVSNDYSFIRYYTRTLYQFQFQEALCQAAKHEGPLHKCDISNSTEAGQKLFNMLRLGKSEPWTLALENVVGAKNMNVRPLLNYFEPLFTWLKDQNKNSFVGWSTDWSPYADQSIKVRISLKSALGDKAYEWNDNEMYLFRCSVAYAMRQYFLKVKNQMILFGEEDVRVANLKPRISFNFFVTAPKNVSDIIPRTEVEKAIRMSRSRINDAFRLNDNSLEFLGIQPTLGDKTHTCPPCPAPELLGGPSVFLFPPKPKDTLMISRTPEVTCVVVDVSHEDPEVKFNWYVDGVEVHNAKTKPREEQYNSTYRVVSVLTVLHQDWLNGKEYKCKVSNKALPAPIEKTISKAKGQPREPQVYTLPPSRDELTKNQVSLTCLVKGFYPSDIAVEWESNGQPENNYKTTPPVLDSDGSFFLYSKLTVDKSRWQQGNVFSCSVMHEALHNHYTQKSLSLSPGK

SEQ ID NO: 84 - protein, 944 aa, synthetic construct
  REGION 1..944: note = ACE2 18-732 T92I Q325P S645C IgG4 wt
QSTIEEQAKTFLDKFNHEAEDLFYQSSLASWNYNTNITEENVQNMNNAGDKWSAFLKEQSTLAQMYPLQEIQNLIVKLQLQALQQNGSSVLSEDKSKRLNTILNTMSTIYSTGKVCNPDNPQECLLLEPGLNEIMANSLDYNERLWAWESWRSEVGKQLRPLYEEYVVLKNEMARANHYEDYGDYWRGDYEVNGVDGYDYSRGQLIEDVEHTFEEIKPLYEHLHAYVRAKLMNAYPSYISPIGCLPAHLLGDMWGRFWTNLYSLTVPFGQKPNIDVTDAMVDQAWDAQRIFKEAEKFFVSVGLPNMTPGFWENSMLTDPGNVQKAVCHPTAWDLGKGDFRILMCTKVTMDDFLTAHHEMGHIQYDMAYAAQPFLLRNGANEGFHEAVGEIMSLSAATPKHLKSIGLLSPDFQEDNETEINFLLKQALTIVGTLPFTYMLEKWRWMVFKGEIPKDQWMKKWWEMKREIVGVVEPVPHDETYCDPASLFHVSNDYSFIRYYTRTLYQFQFQEALCQAAKHEGPLHKCDISNSTEAGQKLFNMLRLGKSEPWTLALENVVGAKNMNVRPLLNYFEPLFTWLKDQNKNSFVGWSTDWSPYADQSIKVRISLKSALGDKAYEWNDNEMYLFRCSVAYAMRQYFLKVKNQMILFGEEDVRVANLKPRISFNFFVTAPKNVSDIIPRTEVEKAIRMSRSRINDAFRLNDNSLEFLGIQPTLGESKYGPPCPPCPAPEFLGGPSVFLFPPKPKDTLMISRTPEVTCVVVDVSQEDPEVQFNWYVDGVEVHNAKTKPREEQFNSTYRVVSVLTVLHQDWLNGKEYKCKVSNKGLPSSIEKTISKAKGQPREPQVYTLPPSQEEMTKNQVSLTCLVKGFYPSDIAVEWESNGQPENNYKTTPPVLDSDGSFFLYSRLTVDKSRWQEGNVFSCSVMHEALHNHYTQKSLSLSLGK

SEQ ID NO: 85 - protein, 942 aa, synthetic construct
  REGION 1..942: note = ACE2 18-732 T92I Q325P S645C IgG1 wt
QSTIEEQAKTFLDKFNHEAEDLFYQSSLASWNYNTNITEENVQNMNNAGDKWSAFLKEQSTLAQMYPLQEIQNLIVKLQLQALQQNGSSVLSEDKSKRLNTILNTMSTIYSTGKVCNPDNPQECLLLEPGLNEIMANSLDYNERLWAWESWRSEVGKQLRPLYEEYVVLKNEMARANHYEDYGDYWRGDYEVNGVDGYDYSRGQLIEDVEHTFEEIKPLYEHLHAYVRAKLMNAYPSYISPIGCLPAHLLGDMWGRFWTNLYSLTVPFGQKPNIDVTDAMVDQAWDAQRIFKEAEKFFVSVGLPNMTPGFWENSMLTDPGNVQKAVCHPTAWDLGKGDFRILMCTKVTMDDFLTAHHEMGHIQYDMAYAAQPFLLRNGANEGFHEAVGEIMSLSAATPKHLKSIGLLSPDFQEDNETEINFLLKQALTIVGTLPFTYMLEKWRWMVFKGEIPKDQWMKKWWEMKREIVGVVEPVPHDETYCDPASLFHVSNDYSFIRYYTRTLYQFQFQEALCQAAKHEGPLHKCDISNSTEAGQKLFNMLRLGKSEPWTLALENVVGAKNMNVRPLLNYFEPLFTWLKDQNKNSFVGWSTDWSPYADQSIKVRISLKSALGDKAYEWNDNEMYLFRCSVAYAMRQYFLKVKNQMILFGEEDVRVANLKPRISFNFFVTAPKNVSDIIPRTEVEKAIRMSRSRINDAFRLNDNSLEFLGIQPTLGDKTHTCPPCPAPELLGGPSVFLFPPKPKDTLMISRTPEVTCVVVDVSHEDPEVKFNWYVDGVEVHNAKTKPREEQYNSTYRVVSVLTVLHQDWLNGKEYKCKVSNKALPAPIEKTISKAKGQPREPQVYTLPPSRDELTKNQVSLTCLVKGFYPSDIAVEWESNGQPENNYKTTPPVLDSDGSFFLYSKLTVDKSRWQQGNVFSCSVMHEALHNHYTQKSLSLSPGK

SEQ ID NO: 86 - protein, 944 aa, synthetic construct
  REGION 1..944: note = ACE2 18-732 T27A T92I Q325P S645C IgG4 wt
QSTIEEQAKAFLDKFNHEAEDLFYQSSLASWNYNTNITEENVQNMNNAGDKWSAFLKEQSTLAQMYPLQEIQNLIVKLQLQALQQNGSSVLSEDKSKRLNTILNTMSTIYSTGKVCNPDNPQECLLLEPGLNEIMANSLDYNERLWAWESWRSEVGKQLRPLYEEYVVLKNEMARANHYEDYGDYWRGDYEVNGVDGYDYSRGQLIEDVEHTFEEIKPLYEHLHAYVRAKLMNAYPSYISPIGCLPAHLLGDMWGRFWTNLYSLTVPFGQKPNIDVTDAMVDQAWDAQRIFKEAEKFFVSVGLPNMTPGFWENSMLTDPGNVQKAVCHPTAWDLGKGDFRILMCTKVTMDDFLTAHHEMGHIQYDMAYAAQPFLLRNGANEGFHEAVGEIMSLSAATPKHLKSIGLLSPDFQEDNETEINFLLKQALTIVGTLPFTYMLEKWRWMVFKGEIPKDQWMKKWWEMKREIVGVVEPVPHDETYCDPASLFHVSNDYSFIRYYTRTLYQFQFQEALCQAAKHEGPLHKCDISNSTEAGQKLFNMLRLGKSEPWTLALENVVGAKNMNVRPLLNYFEPLFTWLKDQNKNSFVGWSTDWSPYADQSIKVRISLKSALGDKAYEWNDNEMYLFRCSVAYAMRQYFLKVKNQMILFGEEDVRVANLKPRISFNFFVTAPKNVSDIIPRTEVEKAIRMSRSRINDAFRLNDNSLEFLGIQPTLGESKYGPPCPPCPAPEFLGGPSVFLFPPKPKDTLMISRTPEVTCVVVDVSQEDPEVQFNWYVDGVEVHNAKTKPREEQFNSTYRVVSVLTVLHQDWLNGKEYKCKVSNKGLPSSIEKTISKAKGQPREPQVYTLPPSQEEMTKNQVSLTCLVKGFYPSDIAVEWESNGQPENNYKTTPPVLDSDGSFFLYSRLTVDKSRWQEGNVFSCSVMHEALHNHYTQKSLSLSLGK

SEQ ID NO: 87 - protein, 942 aa, synthetic construct
  REGION 1..942: note = ACE2 18-732 T27A T92I Q325P S645C IgG1wt
QSTIEEQAKAFLDKFNHEAEDLFYQSSLASWNYNTNITEENVQNMNNAGDKWSAFLKEQSTLAQMYPLQEIQNLIVKLQLQALQQNGSSVLSEDKSKRLNTILNTMSTIYSTGKVCNPDNPQECLLLEPGLNEIMANSLDYNERLWAWESWRSEVGKQLRPLYEEYVVLKNEMARANHYEDYGDYWRGDYEVNGVDGYDYSRGQLIEDVEHTFEEIKPLYEHLHAYVRAKLMNAYPSYISPIGCLPAHLLGDMWGRFWTNLYSLTVPFGQKPNIDVTDAMVDQAWDAQRIFKEAEKFFVSVGLPNMTPGFWENSMLTDPGNVQKAVCHPTAWDLGKGDFRILMCTKVTMDDFLTAHHEMGHIQYDMAYAAQPFLLRNGANEGFHEAVGEIMSLSAATPKHLKSIGLLSPDFQEDNETEINFLLKQALTIVGTLPFTYMLEKWRWMVFKGEIPKDQWMKKWWEMKREIVGVVEPVPHDETYCDPASLFHVSNDYSFIRYYTRTLYQFQFQEALCQAAKHEGPLHKCDISNSTEAGQKLFNMLRLGKSEPWTLALENVVGAKNMNVRPLLNYFEPLFTWLKDQNKNSFVGWSTDWSPYADQSIKVRISLKSALGDKAYEWNDNEMYLFRCSVAYAMRQYFLKVKNQMILFGEEDVRVANLKPRISFNFFVTAPKNVSDIIPRTEVEKAIRMSRSRINDAFRLNDNSLEFLGIQPTLGDKTHTCPPCPAPELLGGPSVFLFPPKPKDTLMISRTPEVTCVVVDVSHEDPEVKFNWYVDGVEVHNAKTKPREEQYNSTYRVVSVLTVLHQDWLNGKEYKCKVSNKALPAPIEKTISKAKGQPREPQVYTLPPSRDELTKNQVSLTCLVKGFYPSDIAVEWESNGQPENNYKTTPPVLDSDGSFFLYSKLTVDKSRWQQGNVFSCSVMHEALHNHYTQKSLSLSPGK